European Patent Application EP 4 406 549 A2, published July 31, 2024. Title: Human-derived anti-huntingtin (HTT) antibodies and uses thereof. Applicant: Neurimmune Holding AG. The sequence listing filed with the application follows.

SEQUENCE LISTING (202 sequences)

SEQ ID NO: 1 - DNA, 369 bp, Homo sapiens
  V_region 91..105: note = complementarity determining region (CDR) VH-CDR1
  V_region 148..198: note = complementarity determining region (CDR) VH-CDR2
  V_region 295..336: note = complementarity determining region (CDR) VH-CDR3
  source 1..369: mol_type = other DNA
  CDS 1..369: note = NI-302.33C11-VH variable heavy chain (VH) sequence
gaggtgcagctggtggagtctgggggaggcgttgtccagcctgggaactccctgagactctcctgtgcagcgtctggattcaggttcagtgactttggcatgcactgggtccgccaggctccaggcaagggactggagtggctggcacttatatggtatgatggagggtataagtactatgcagactccgtgaagggccgattcaccatctccagagacaattccaagaatacgatgtttctacaaatgaacagcctgagagccgaggacacggctgtttattactgtgcgacccacctagaatattgcagtagaaccacctgctatctcggccactggggccagggaaccctggtcaccgtctcctcg

SEQ ID NO: 2 - protein, 123 aa, Homo sapiens
EVQLVESGGGVVQPGNSLRLSCAASGFRFSDFGMHWVRQAPGKGLEWLALIWYDGGYKYYADSVKGRFTISRDNSKNTMFLQMNSLRAEDTAVYYCATHLEYCSRTTCYLGHWGQGTLVTVSS

SEQ ID NO: 3 - DNA, 321 bp, Homo sapiens
  V_region 70..102: note = complementarity determining region (CDR) VK-CDR1
  V_region 148..168: note = complementarity determining region (CDR) VK-CDR2
  V_region 265..291: note = complementarity determining region (CDR) VK-CDR3
  source 1..321: mol_type = other DNA
  CDS 1..321: note = NI-302.33C11-VK variable light-kappa chain (VK) sequence
gacatccagttgacccagtctccgtccttcctatctgcgtctgtgggagacacagtcaccttcacttgccgggccagtcagggcattagcgattatttagcctggtttcagcagaaaccagggattgcccctaagctcctgatctatgctgcgtccactttgcaaaccggggtcccatcaaggttcagcggcagtggatctgggacagaattcactctcacaatccgcagcctgcagtctgaagattttggaacttattactgtcagcagcttaaaacttacccgtacacttttggccaggggaccaaggtggaaatcaaa

SEQ ID NO: 4 - protein, 107 aa, Homo sapiens
DIQLTQSPSFLSASVGDTVTFTCRASQGISDYLAWFQQKPGIAPKLLIYAASTLQTGVPSRFSGSGSGTEFTLTIRSLQSEDFGTYYCQQLKTYPYTFGQGTKVEIK

SEQ ID NO: 5 - DNA, 357 bp, Homo sapiens
  V_region 91..105: note = complementarity determining region (CDR) VH-CDR1
  V_region 148..198: note = complementarity determining region (CDR) VH-CDR2
  V_region 295..324: note = complementarity determining region (CDR) VH-CDR3
  source 1..357: mol_type = other DNA
  CDS 1..357: note = NI-302.63F3 VH variable heavy chain (VH) sequence
caggtgcagctggtgcaatctgggtctgcgttcaagaagcctgggacctcagtgaaagtttcctgcaaggcctctggatacaccttcgagacccgttctatgaactgggtgcgacaggcccctggacaagggcttgaatacatgggatggatcaacaccaacactggcaaccgcacgtatgtccaggccttcagaggacgatttgtcttctccttggacacctctgtcagcacggcatatctgcagatcagcaacttaaagactgaggacactgccgtgtattactgtgcgagaggggcaggtgggggatattggttcgactcctggggccagggaaccctggtcaccgtctcctcg

SEQ ID NO: 6 - protein, 119 aa, Homo sapiens
QVQLVQSGSAFKKPGTSVKVSCKASGYTFETRSMNWVRQAPGQGLEYMGWINTNTGNRTYVQAFRGRFVFSLDTSVSTAYLQISNLKTEDTAVYYCARGAGGGYWFDSWGQGTLVTVSS

SEQ ID NO: 7 - DNA, 339 bp, Homo sapiens
  V_region 70..120: note = complementarity determining region (CDR) VK-CDR1
  V_region 166..186: note = complementarity determining region (CDR) VK-CDR2
  V_region 283..309: note = complementarity determining region (CDR) VK-CDR3
  source 1..339: mol_type = other DNA
  CDS 1..339: note = NI-302.63F3 VK variable light-kappa chain (VK) sequence
gacatccagatgacccagtctccagactccctggctgtgtctctgggcgagagggccaccatcaactgcaagtccaatcagagtcttttctacagttccaacaataacaactacttagcttggtaccagcacaaatccggacagcctcctaagctgctcgtttactggggatctacccgggaatccggggtccctgaccgcttcagtggcagcgggtctgggactgacttcactctcaccatcagtagcctgcaggctgaggatgttgcaatttattactgtcaccaatattatcataatccgtacacttttggccaggggaccaagctggagatcaaa

SEQ ID NO: 8 - protein, 113 aa, Homo sapiens
DIQMTQSPDSLAVSLGERATINCKSNQSLFYSSNNNNYLAWYQHKSGQPPKLLVYWGSTRESGVPDRFSGSGSGTDFTLTISSLQAEDVAIYYCHQYYHNPYTFGQGTKLEIK

SEQ ID NO: 9 - DNA, 363 bp, Homo sapiens
  V_region 91..105: note = complementarity determining region (CDR) VH-CDR1
  V_region 148..198: note = complementarity determining region (CDR) VH-CDR2
  V_region 295..330: note = complementarity determining region (CDR) VH-CDR3
  source 1..363: mol_type = other DNA
  CDS 1..363: note = NI-302.35C1 VH variable heavy chain (VH) sequence
gaggtgcagctggtggagtctgggggaaacttggtacagccgggggggtccctgagactctcctgtactgcctctggattcacctttagtataacggccctgagttgggtccgccaggctccagaaaaggggccgcagtgggtctcagcaatcactggaaatgcttatgggacatactacgcagactccgtgaagggccggttcaccatttccagagacaacgccaagaacacactgtacttgcaaatgaacggcctgagagccgaggacacggccatctattactgtgtgaaaggaattgcctccgatagtagtggttattctgccttctggggcccgggcaccctggtcaccgtctcctcg

SEQ ID NO: 10 - protein, 121 aa, Homo sapiens
EVQLVESGGNLVQPGGSLRLSCTASGFTFSITALSWVRQAPEKGPQWVSAITGNAYGTYYADSVKGRFTISRDNAKNTLYLQMNGLRAEDTAIYYCVKGIASDSSGYSAFWGPGTLVTVSS

SEQ ID NO: 11 - DNA, 321 bp, Homo sapiens
  V_region 70..102: note = complementarity determining region (CDR) VK-CDR1
  V_region 148..168: note = complementarity determining region (CDR) VK-CDR2
  V_region 265..291: note = complementarity determining region (CDR) VK-CDR3
  source 1..321: mol_type = other DNA
  CDS 1..321: note = NI-302.35C1 VK variable light -kappa chain (VK) sequence
gaaattgtgctgactcagtctccagccaccctgtctttgtctccaggggaaagagccaccctctcctgcagggccagtcaaagtgttgacaaccagtttgcctggtaccaacagaaacctggccaggctcccaggctcctcatttatgatgcatccaggagggcccctggcatcccagacaggttcagtggcagtgggtctgggacagacttcactctcaccattagcagcctagagcctgaagatttcgcaatttattactgtcagcatcgttacacctggctctacacttttggccaggggacacgactggagattaaa

SEQ ID NO: 12 - protein, 107 aa, Homo sapiens
EIVLTQSPATLSLSPGERATLSCRASQSVDNQFAWYQQKPGQAPRLLIYDASRRAPGIPDRFSGSGSGTDFTLTISSLEPEDFAIYYCQHRYTWLYTFGQGTRLEIK

SEQ ID NO: 13 - DNA, 357 bp, Homo sapiens
  V_region 91..105: note = complementarity determining region (CDR) VH-CDR1
  V_region 148..195: note = complementarity determining region (CDR) VH-CDR2
  V_region 292..324: note = complementarity determining region (CDR) VH-CDR3
  source 1..357: mol_type = other DNA
  CDS 1..357: note = NI-302.31F11 VH variable heavy chain (VH) sequence
gaggtgcagctggtggagtccggaggaggcttgatccagccgggggggtccctgagactctcctgtgcagcctctgggttcaccgtcagcagcacctacatgagttgggtccgccaggctccagggaaggggcttgagtgcgtctcagttatttttagtggcgctgacacatattacgcagactccgtgaagggccgattcaccgtctccagagacaattccaagaacacactgtttcttcagatgaacagcctgagagtcgaggacacggccacatattactgtgtgagacattattatggttcagaccttccatctgacttctggggccagggcaccctggtcaccgtctcctcg

SEQ ID NO: 14 - protein, 119 aa, Homo sapiens
EVQLVESGGGLIQPGGSLRLSCAASGFTVSSTYMSWVRQAPGKGLECVSVIFSGADTYYADSVKGRFTVSRDNSKNTLFLQMNSLRVEDTATYYCVRHYYGSDLPSDFWGQGTLVTVSS

SEQ ID NO: 15 - DNA, 336 bp, Homo sapiens
  V_region 70..117: note = complementarity determining region (CDR) VK-CDR1
  V_region 163..183: note = complementarity determining region (CDR) VK-CDR2
  V_region 280..306: note = complementarity determining region (CDR) VK-CDR3
  source 1..336: mol_type = other DNA
  CDS 1..336: note = NI-302.31F11 VK variable light-kappa chain (VK) sequence
gatgttgtgatgactcagtctccactctccctgcccgtcgcccctggagagccggcctccatctcctgcaggtctagtcagagcctcctatacagtaatggatacaactatttggattggtacctgcagaagccagggaagcctccacagctcctggtctatttgggttctgatcgggcctccggggtccctgacaggttcagtggcagtggatcaggcaaagattttacactgaacatcagcagagtggaggctgaggatgttggggtttattactgcatgcaaggtctacaaagtccgtggacgttcggccaagggaccaagctggagatcaaa

SEQ ID NO: 16 - protein, 112 aa, Homo sapiens
DVVMTQSPLSLPVAPGEPASISCRSSQSLLYSNGYNYLDWYLQKPGKPPQLLVYLGSDRASGVPDRFSGSGSGKDFTLNISRVEAEDVGVYYCMQGLQSPWTFGQGTKLEIK

SEQ ID NO: 17 - DNA, 354 bp, Homo sapiens
  V_region 91..105: note = complementarity determining region (CDR) VH-CDR1
  V_region 148..198: note = complementarity determining region (CDR) VH-CDR2
  V_region 295..321: note = complementarity determining region (CDR) VH-CDR3
  source 1..354: mol_type = other DNA
  CDS 1..354: note = NI-302.2A2 VH variable heavy chain (VH) sequence
gaggtgcagctggtggagtctgggggaggcttggtccagcctggggggtccctgagactctcctgtgcagcctctggattcacctttagtacctattggatgaactgggtccgccaggctccagggaaggggctggagtgggtggccaacataaaaccagatggaagtgacaaatactatgtggactctgtgaagggccgattcaccatctccagagacaacgccaagaactcactgtatctgcaaatgaacagcctgagagacgaggacacggctgtgtattactgtgcgagaggggacggcagtggctggaacgtctactggggccagggaaccctggtcaccgtctcctcg

SEQ ID NO: 18 - protein, 118 aa, Homo sapiens
EVQLVESGGGLVQPGGSLRLSCAASGFTFSTYWMNWVRQAPGKGLEWVANIKPDGSDKYYVDSVKGRFTISRDNAKNSLYLQMNSLRDEDTAVYYCARGDGSGWNVYWGQGTLVTVSS

SEQ ID NO: 19 - DNA, 345 bp, Homo sapiens
  V_region 70..129: note = complementarity determining region (CDR) VK-CDR1
  V_region 175..195: note = complementarity determining region (CDR) VK-CDR2
  V_region 292..315: note = complementarity determining region (CDR) VK-CDR3
  source 1..345: mol_type = other DNA
  CDS 1..345: note = NI-302.2A2 VK variable light-kappa chain (VK) sequence
gacatccagatgacccagtctccagactccctggctgtgtctctgggcgagagggccaccatcaactgcaagtccagccagagtcttttatacacctccaaaaataaggacagtaagaactacttaggttggtaccagcagaaaccaggacagcctcctaagctgctcatttactgggcatctacccgggaatccggggtccctgaccgattcagtggcagcgggtctgggacagatttcactctcaccatcagcagcctgcaggctgaggatgtggcagtttattactgtcagcagtattatactactcctcagttcggcggagggaccaaggtggagatcaaa

SEQ ID NO: 20 - protein, 115 aa, Homo sapiens
DIQMTQSPDSLAVSLGERATINCKSSQSLLYTSKNKDSKNYLGWYQQKPGQPPKLLIYWASTRESGVPDRFSGSGSGTDFTLTISSLQAEDVAVYYCQQYYTTPQFGGGTKVEIK

SEQ ID NO: 21 - DNA, 369 bp, Homo sapiens
  V_region 91..105: note = complementarity determining region (CDR) VH-CDR1
  V_region 148..198: note = complementarity determining region (CDR) VH-CDR2
  V_region 295..336: note = complementarity determining region (CDR) VH-CDR3
  source 1..369: mol_type = other DNA
  CDS 1..369: note = NI-302.6N9 VH variable heavy chain (VH) sequence
gaggtgcagctggtggagtctgggggagacttggtgcagcctggggggtccctgagactctcctgtgtagtctctggattcacctttagtagttatgccatgacctgggtccgccaggctccagggaaggggctggcctgggtctcaacaattagtgctactggtggtagtacattctacacagactccgtgaggggccggttcaccatctcccgagacaattccaagaacacactgtatctgcaaatgaatagcctgagaaccgacgacacggccatatattattgtgtgaaagatctatttggagtggacacctcctactacggtatggacgtctggggccaagggaccacggtcaccgtctcctcg

SEQ ID NO: 22 - protein, 123 aa, Homo sapiens
EVQLVESGGDLVQPGGSLRLSCVVSGFTFSSYAMTWVRQAPGKGLAWVSTISATGGSTFYTDSVRGRFTISRDNSKNTLYLQMNSLRTDDTAIYYCVKDLFGVDTSYYGMDVWGQGTTVTVSS

SEQ ID NO: 23 - DNA, 324 bp, Homo sapiens
  V_region 70..105: note = complementarity determining region (CDR) VK-CDR1
  V_region 151..171: note = complementarity determining region (CDR) VK-CDR2
  V_region 268..294: note = complementarity determining region (CDR) VK-CDR3
  source 1..324: mol_type = other DNA
  CDS 1..324: note = NI-302.6N9 VK variable light-kappa chain (VK) sequence
gaaattgtgttgacgcagtctccaggcaccctgtctttgtctccaggggaaagagccaccctctcctgcaggcccagtcagagtgtcagcggcaggtatgtggcctggtatcagcagaaacctggccaggctcccaggctcctcttctatgctgcatccaacagggccattggcatcccagacaggttcagtggcagtgggtctgggacagacttcactctcaccatcagcagactggagcctgaagattttgcagtgtattactgtcagcactatggtgcctcatcgtacacttttggcccggggaccaaagtggatatcaaa

SEQ ID NO: 24 - protein, 108 aa, Homo sapiens
EIVLTQSPGTLSLSPGERATLSCRPSQSVSGRYVAWYQQKPGQAPRLLFYAASNRAIGIPDRFSGSGSGTDFTLTISRLEPEDFAVYYCQHYGASSYTFGPGTKVDIK

SEQ ID NO: 25 - DNA, 360 bp, Homo sapiens
  V_region 91..105: note = complementarity determining region (CDR) VH-CDR1
  V_region 148..186: note = complementarity determining region (CDR) VH-CDR2
  V_region 295..327: note = complementarity determining region (CDR) VH-CDR3
  source 1..360: mol_type = other DNA
  CDS 1..360: note = NI-302.74C11 VH variable heavy chain (VH) sequence
gaggtgcagctggtgcagtctgggactgaggtgcagaagcctggggcctcagtaaaagtctcctgcaaggcttctggatacagtttcaccggctactttttgcactgggtacgacaggcccctggacaagggcttgagtggatggggtggatcaaccctaacagtggtgacacaaactatgcagagaagtttcggggcagaatcatcatgaccagggacacgtctgtcagcacagcccacatggagttgagcagcctgagatttgacgacacggccctatattactgtacgagagaggcccctgacccgggcgctgagacggacgtctggggccaagggaccacggtcaccgtctcctcg

SEQ ID NO: 26 - protein, 120 aa, Homo sapiens
EVQLVQSGTEVQKPGASVKVSCKASGYSFTGYFLHWVRQAPGQGLEWMGWINPNSGDTNYAEKFRGRIIMTRDTSVSTAHMELSSLRFDDTALYYCTREAPDPGAETDVWGQGTTVTVSS

SEQ ID NO: 27 - DNA, 321 bp, Homo sapiens
  V_region 67..99: note = complementarity determining region (CDR) VL-CDR1
  V_region 145..165: note = complementarity determining region (CDR) VL-CDR2
  V_region 262..291: note = complementarity determining region (CDR) VL-CDR3
  source 1..321: mol_type = other DNA
  CDS 1..321: note = NI-302.74C11 VL variable light chain (VL) sequence
cagtctgtgctgactcagccaccctcggtgtcagtgtccccaggacagacggccaggatcacctgctctggagatgcagtgccaaagcagtatatttattggtaccagcagaagccaggccaggcccctattctggtgatatataaagacactcagaggccttcagggatccctgagcgattctctggctccaactcagggacaacagtcacgttgaccataactggcgtccaggcagacgacgagggtgactattactgtcaatcagcagacagtagtgctacttgggtgttcggcggagggaccaaattgaccgtccta

SEQ ID NO: 28 - protein, 107 aa, Homo sapiens
QSVLTQPPSVSVSPGQTARITCSGDAVPKQYIYWYQQKPGQAPILVIYKDTQRPSGIPERFSGSNSGTTVTLTITGVQADDEGDYYCQSADSSATWVFGGGTKLTVL

SEQ ID NO: 29 - DNA, 360 bp, Homo sapiens
  V_region 91..105: note = complementarity determining region (CDR) VH-CDR1
  V_region 148..201: note = complementarity determining region (CDR) VH-CDR2
  V_region 298..327: note = complementarity determining region (CDR) VH-CDR3
  source 1..360: mol_type = other DNA
  CDS 1..360: note = NI-302.15F9 VH variable heavy chain (VH) sequence
gaggtgcagctggtggagtctgggggaggcctggtcacgccgggggggtccctgagactctcgtgtgaggcctctggatttctcttcaagaattctagcatgaactgggtccgtcagactccggggaaggggctggagtgggtctcgtccattgacacttctgctacaaattataagtattatgcagactctgtgaagggccgatttaccatctccagggatgacgccaccaactctctctatctgcaaatgaatagcctgcgagccgacgacacggctacttattactgtgcgcgaggttattataccccccgggactttgactactggggccagggcaccctggtcaccgtctcctcg

SEQ ID NO: 30 - protein, 120 aa, Homo sapiens
EVQLVESGGGLVTPGGSLRLSCEASGFLFKNSSMNWVRQTPGKGLEWVSSIDTSATNYKYYADSVKGRFTISRDDATNSLYLQMNSLRADDTATYYCARGYYTPRDFDYWGQGTLVTVSS

SEQ ID NO: 31 - DNA, 336 bp, Homo sapiens
  V_region 70..117: note = complementarity determining region (CDR) VK-CDR1
  V_region 163..183: note = complementarity determining region (CDR) VK-CDR2
  V_region 280..306: note = complementarity determining region (CDR) VK-CDR3
  source 1..336: mol_type = other DNA
  CDS 1..336: note = NI-302.15F9 VK variable light-kappa chain (VK) sequence
gatgttgtgatgactcagtctccacagaccctgtccgtcagccttggacaggcggcctccatctcctgcaggtcgagtcaaagcctcttgtatcgtgataacaacacatacttgaattggtttcaccagaggccaggccaatctccaaggcgcctcatttatagggcttctgaccgggactctggggtcccagacagattcagcggcggtgggtcaggcactgatttcacattgaaaatcagtggagtggaggctgaagatgttggcacttattactgcatgcaaggaacacactggcctcggacgttcggccaagggaccaaggtggagatcaaa

SEQ ID NO: 32 - protein, 112 aa, Homo sapiens
DVVMTQSPQTLSVSLGQAASISCRSSQSLLYRDNNTYLNWFHQRPGQSPRRLIYRASDRDSGVPDRFSGGGSGTDFTLKISGVEAEDVGTYYCMQGTHWPRTFGQGTKVEIK

SEQ ID NO: 33 - DNA, 357 bp, Homo sapiens
  V_region 91..105: note = complementarity determining region (CDR) VH-CDR1
  V_region 148..195: note = complementarity determining region (CDR) VH-CDR2
  V_region 292..324: note = complementarity determining region (CDR) VH-CDR3
  source 1..357: mol_type = other DNA
  CDS 1..357: note = NI-302.39G12 VH variable heavy chain (VH) sequence
gaggtgcagctggtgcagtctgggggaggcttggtccacccttgggggtccctgagactctcctgtgcagcctctggattcagcgtctctaattacgccataacttgggtccgccgggctccagggaaggggctgcaatatatttcagtaatttatcgtgatggcaggacatactacggagactccgtgaggggccgcttcaccatctctagggacgattccaagaacactctctatcttcaaatgaacagcctgagatttgaggacacggctgtgtattactgtgcgagagcgcacggccaatattactatggtgtggacgtctggggccaagggaccacggtcaccgtctcctcg

SEQ ID NO: 34 - protein, 119 aa, Homo sapiens
EVQLVQSGGGLVHPWGSLRLSCAASGFSVSNYAITWVRRAPGKGLQYISVIYRDGRTYYGDSVRGRFTISRDDSKNTLYLQMNSLRFEDTAVYYCARAHGQYYYGVDVWGQGTTVTVSS

SEQ ID NO: 35 - DNA, 333 bp, Homo sapiens
  V_region 70..117: note = complementarity determining region (CDR) VK-CDR1
  V_region 163..183: note = complementarity determining region (CDR) VK-CDR2
  V_region 280..306: note = complementarity determining region (CDR) VK-CDR3
  source 1..333: mol_type = other DNA
  CDS 1..333: note = NI-302.39G12 VK variable light-kappa chain (VK) sequence
gatgttgtgatgactcagtctccactctccctgtccgtcagccctggagagccggcctccatctcctgcaggtctagtcagagcctcctacatagtaatggatacaactatttggattggtaccggcagaaaccagggcagtctccacagctcctgatctatttgagttctaatcggccctccggggtccctgataggttcagtgccagtggatcaggcacagagttcacactgcaaatcagcagagtggaggctgaggatgttggggtttattactgcatgcaatctctgcaaacgttcactttcggcggagggaccaaagtggatatcaaa

SEQ ID NO: 36 - protein, 111 aa, Homo sapiens
DVVMTQSPLSLSVSPGEPASISCRSSQSLLHSNGYNYLDWYRQKPGQSPQLLIYLSSNRPSGVPDRFSASGSGTEFTLQISRVEAEDVGVYYCMQSLQTFTFGGGTKVDIK

SEQ ID NO: 37 - DNA, 363 bp, Homo sapiens
  V_region 91..105: note = complementarity determining region (CDR) VH-CDR1
  V_region 148..195: note = complementarity determining region (CDR) VH-CDR2
  V_region 292..330: note = complementarity determining region (CDR) VH-CDR3
  source 1..363: mol_type = other DNA
  CDS 1..363: note = NI-302.11A4 VH variable heavy chain (VH) sequence
gaggtgcagctggtggagtctggaggaggcttgatccagccgggggggtccctgagactctcctgtgcagcctctgggttccccgtcagtagcagttacatgagctgggtccgccaggctccaggagaggggctggagtgggtctcagttctttatagagacggtgacacatactacgcagactccgtgcagggccgattcaccatctccagagacaattcccagaacacgttctatcttcaaatgaacagcctgaaagccgaggacacggccgtgtattactgtgcgggtgatagaaggtcgtcacactactattacggtatggacgtctggggccaggggaccacggtcaccgtctcctcg

SEQ ID NO: 38 - protein, 121 aa, Homo sapiens
EVQLVESGGGLIQPGGSLRLSCAASGFPVSSSYMSWVRQAPGEGLEWVSVLYRDGDTYYADSVQGRFTISRDNSQNTFYLQMNSLKAEDTAVYYCAGDRRSSHYYYGMDVWGQGTTVTVSS

SEQ ID NO: 39 - DNA, 321 bp, Homo sapiens
  V_region 70..105: note = complementarity determining region (CDR) VK-CDR1
  V_region 151..171: note = complementarity determining region (CDR) VK-CDR2
  V_region 268..291: note = complementarity determining region (CDR) VK-CDR2
  source 1..321: mol_type = other DNA
  CDS 1..321: note = NI-302.11A4 VK variable light-kappa chain (VK) sequence
gaaattgtgatgacacagtctccaggcaccctgtctttgtctccaggagaaagagccaccctctcctgcagggccagtcagagtgttagcagcagctacttcgcctggtaccaacaaaaacctggccaggctcccaggctcctcatctatggtacgtcccgcagggccactgccatcccagacaggttcagtggcagtgggtctgggacagacttcactctcaccatcagcagactggagcctgaagattttgcagtgtattactgtcaacagtatggtagctcgtggacgttcggcccagggaccaaggtggagatcaaa

SEQ ID NO: 40 - protein, 107 aa, Homo sapiens
EIVMTQSPGTLSLSPGERATLSCRASQSVSSSYFAWYQQKPGQAPRLLIYGTSRRATAIPDRFSGSGSGTDFTLTISRLEPEDFAVYYCQQYGSSWTFGPGTKVEIK

SEQ ID NO: 41 - DNA, 357 bp, Homo sapiens
  V_region 91..105: note = complementarity determining region (CDR) VH-CDR1
  V_region 148..195: note = complementarity determining region (CDR) VH-CDR2
  V_region 292..324: note = complementarity determining region (CDR) VH-CDR3
  source 1..357: mol_type = other DNA
  CDS 1..357: note = NI-302.22H9 VH variable heavy chain (VH) sequence
gaggtgcagctggtggagtctgggggaggcttggtccacccttgggggtccctgagagtctcctgtgcagcctctggattcagcgtctctaattacgccataacttgggtccgccaggctccagggaaggggctggaatatatttcagtgatttatcgtgatggcaggacatactacggagactccgtgaggggccgcttcaccatctctagggacgattccaagaacactatctatcttcaaatgaacagcctgagatttgaggacacggctgtgtattactgtgcgagagcgcacggccaatattattatggtgtggacgtctggggccaagggaccacggtcaccgtctcctcg

SEQ ID NO: 42 - protein, 119 aa, Homo sapiens
EVQLVESGGGLVHPWGSLRVSCAASGFSVSNYAITWVRQAPGKGLEYISVIYRDGRTYYGDSVRGRFTISRDDSKNTIYLQMNSLRFEDTAVYYCARAHGQYYYGVDVWGQGTTVTVSS

SEQ ID NO: 43 - DNA, 333 bp, Homo sapiens
  V_region 70..117: note = complementarity determining region (CDR) VK-CDR1
  V_region 163..183: note = complementarity determining region (CDR) VK-CDR2
  V_region 280..303: note = complementarity determining region (CDR) VK-CDR3
  source 1..333: mol_type = other DNA
  CDS 1..333: note = NI-302.22H9 VK variable light-kappa chain (VK) sequence
gatgttgtgatgactcagtctccactctccctgtccgtcagccctggagagccggcctccatctcctgcaggtctagtcagagcctcctacatagtaatggatacaactatttggattggtaccggcagaaaccagggcagtctccacaactcctgatctatttgaattctaatcgggcctccggggtccctgataggttcagtggcagtggatcaggcacagagttcacactgacaatcagcagagtggaggctgaggatgttggggtttattactgcatgcaatctctgcaaacgttcactttcggcggagggaccaaggtggagatcaaa

SEQ ID NO: 44 - protein, 111 aa, Homo sapiens
DVVMTQSPLSLSVSPGEPASISCRSSQSLLHSNGYNYLDWYRQKPGQSPQLLIYLNSNRASGVPDRFSGSGSGTEFTLTISRVEAEDVGVYYCMQSLQTFTFGGGTKVEIK

SEQ ID NO: 45 - DNA, 357 bp, Homo sapiens
  V_region 91..105: note = complementarity determining region (CDR) VH-CDR1
  V_region 148..198: note = complementarity determining region (CDR) VH-CDR2
  V_region 295..324: note = complementarity determining region (CDR) VH-CDR3
  source 1..357: mol_type = other DNA
  CDS 1..357: note = NI-302.44D7 VH variable heavy chain (VH) sequence
gaggtgcagctggtgcagtctgggggaggcttggtacagcctggggggtccctgagactctcctgtgcagcctctggattcacctttagcagctatgccatgagttgggtccgccaggctccagggaaggggctggagtgggtctcaggtattggttatagtgatactagcacatattacgcagactccgtgaagggccgcttcaccgtctccagagacatttccaagaacacgctgtatctgcaaatgaatagcctgagggccgaggacacggccgtatattactgcgcgaaaggtaccagggactattacggtatggacgtctggggccaagggacaatggtcaccgtctcttcg

SEQ ID NO: 46 - protein, 119 aa, Homo sapiens
EVQLVQSGGGLVQPGGSLRLSCAASGFTFSSYAMSWVRQAPGKGLEWVSGIGYSDTSTYYADSVKGRFTVSRDISKNTLYLQMNSLRAEDTAVYYCAKGTRDYYGMDVWGQGTMVTVSS

SEQ ID NO: 47 - DNA, 330 bp, Homo sapiens
  V_region 67..108: note = complementarity determining region (CDR) VL-CDR1
  V_region 192..198: note = complementarity determining region (CDR) VL-CDR2
  V_region 271..300: note = complementarity determining region (CDR) VL-CDR3
  source 1..330: mol_type = other DNA
  CDS 1..330: note = NI-302.44D7 VL variable light chain (VL) sequence
cagactgtggtgactcaggagccatcgttctcagtgtcccctggagggacagtcacactcacttgtggcttgagttctggctcagtttctactagttactaccccagctggtaccagcagaccccaggccgggctccacgcacgctcatctacagcacaaacactcgctcttctggggtccctgatcgcttctctggctccatccttgggaacaaggctgccctcaccatcacgggggcccaggcagatgatgaatctgattattactgtgtgctgtttatgggtagtggcattggggtgttcggcggagggaccaggctgaccgtccta

SEQ ID NO: 48 - protein, 110 aa, Homo sapiens
QTVVTQEPSFSVSPGGTVTLTCGLSSGSVSTSYYPSWYQQTPGRAPRTLIYSTNTRSSGVPDRFSGSILGNKAALTITGAQADDESDYYCVLFMGSGIGVFGGGTRLTVL

SEQ ID NO: 49 - DNA, 357 bp, Homo sapiens
  V_region 91..105: note = complementarity determining region (CDR) VH-CDR1
  V_region 148..192: note = complementarity determining region (CDR) VH-CDR2
  V_region 292..324: note = complementarity determining region (CDR) VH-CDR3
  source 1..357: mol_type = other DNA
  CDS 1..357: note = NI-302.37C12 VH variable heavy chain (VH) sequence
gaggtgcagctggtggagtctggtggaggcttggtccagcctggggggtccctgagactctcttgtgttgcctctgcactcaccgtcactaacagccaaatgacctgggtccgccgggctccagggagggggttggagtgggtctcagttatttacaccagtggtagtgcatactacgcagactccgtgaagggcagattcaccatctccagagacaattccaagaacacagtgtttcttcaaatgaacagcctgagagtcgaagacacggctgtgtattactgtgcgaaaggcccatcagcctattattacggtttggacctttggggccaagggaccacggtcaccgtctcctcg

SEQ ID NO: 50 - protein, 119 aa, Homo sapiens
EVQLVESGGGLVQPGGSLRLSCVASALTVTNSQMTWVRRAPGRGLEWVSVIYTSGSAYYADSVKGRFTISRDNSKNTVFLQMNSLRVEDTAVYYCAKGPSAYYYGLDLWGQGTTVTVSS

SEQ ID NO: 51 - DNA, 333 bp, Homo sapiens
  V_region 70..117: note = complementarity determining region (CDR) VK-CDR1
  V_region 163..183: note = complementarity determining region (CDR) VK-CDR2
  V_region 280..303: note = complementarity determining region (CDR) VK-CDR3
  source 1..333: mol_type = other DNA
  CDS 1..333: note = NI-302.37C12 VK variable light-kappa chain (VK) sequence
gatattgtgatgactcaatcaccactctccctgcccgtcacccctggagagccggcctccatctcctgcaggtctagtcagagcctcctgcatagtaatggatacaactatttggattggtacctgcagaagccggggcagtctccacagctcctgatctatttgggttctactcgggcctccggggtccctgacaggttcagtggcagtggatcaggcacagattttacactgaagatcagcagagtggaggctgaggatgttggggtttattactgcatgcaaggtctacagacgtacacttttggccaggggaccaagctggagatcaaa

SEQ ID NO: 52 - protein, 111 aa, Homo sapiens
DIVMTQSPLSLPVTPGEPASISCRSSQSLLHSNGYNYLDWYLQKPGQSPQLLIYLGSTRASGVPDRFSGSGSGTDFTLKISRVEAEDVGVYYCMQGLQTYTFGQGTKLEIK

SEQ ID NO: 53 - DNA, 378 bp, Homo sapiens
  V_region 91..105: note = complementarity determining region (CDR) VH-CDR1
  V_region 148..213: note = complementarity determining region (CDR) VH-CDR2
  V_region 295..345: note = complementarity determining region (CDR) VH-CDR3
  source 1..378: mol_type = other DNA
  CDS 1..378: note = NI-302.55D8 VH variable heavy chain (VH) sequence
caggtgcagctggtgcagtctgggtctgaggtgaagaagcctggggcctcagtgaaggtctcctgcaaggcttctggatacaccttcaccgactactatatacactgggtgcgacaggcccctggacaagggcttgagtggatgggacggatcaaccctaacaatggtggcacaaactatgcacagaactttcagggctgggtcaccatgaccagggacacgtccatcagcacagcctacatggagctcagcagactgagatctgacgacacggccgtctattactgtgcgagagtggggggcgagctgctacgagaaggcggctatcactactacatggacgtctggggcaaggggaccacggtcaccgtctcctcg

SEQ ID NO: 54 - protein, 126 aa, Homo sapiens
QVQLVQSGSEVKKPGASVKVSCKASGYTFTDYYIHWVRQAPGQGLEWMGRINPNNGGTNYAQNFQGWVTMTRDTSISTAYMELSRLRSDDTAVYYCARVGGELLREGGYHYYMDVWGKGTTVTVSS

SEQ ID NO: 55 - DNA, 336 bp, Homo sapiens
  V_region 67..108: note = complementarity determining region (CDR) VL-CDR1
  V_region 154..174: note = complementarity determining region (CDR) VL-CDR2
  V_region 271..306: note = complementarity determining region (CDR) VL-CDR3
  source 1..336: mol_type = other DNA
  CDS 1..336: note = NI-302.55D8 VL variable light chain (VL) sequence
cagtctgtgttgacgcagccgccctcagtgtctggggccccagggcagagggtcaccatctcctgcactgggaacagctccaacatcggggcaggttatgatgtacactggtaccagcagcttccaggaacagcccccaaactcctcatctttgataataccaatcggccctcaggggtccctgaccgattctctggctccaagtctggcacctcagcctccctggccatcactgggctccaggctgaggatgaggctaattatcactgccagtcctatgacaacagcctgagtggttcttgggtgttcggcggagggaccaagctgaccgtccta

SEQ ID NO: 56 - protein, 112 aa, Homo sapiens
QSVLTQPPSVSGAPGQRVTISCTGNSSNIGAGYDVHWYQQLPGTAPKLLIFDNTNRPSGVPDRFSGSKSGTSASLAITGLQAEDEANYHCQSYDNSLSGSWVFGGGTKLTVL

SEQ ID NO: 57 - DNA, 369 bp, Homo sapiens
  V_region 91..105: note = complementarity determining region (CDR) VH-CDR1
  V_region 148..198: note = complementarity determining region (CDR) VH-CDR2
  V_region 295..336: note = complementarity determining region (CDR) VH-CDR3
  source 1..369: mol_type = other DNA
  CDS 1..369: note = NI-302.7A8 VH variable heavy chain (VH) sequence
gaggtgcagctggtggagtctgggggaggctcggtccagcctggggggtccctgagactctcctgtgtagcctctggattcatatttagaaacagttggatgacctgggtccgccaggatccagggaaggggctggagtgggtggccaacataaaggaagatggaagtcggacatactatgtggactctgtgaagggccgattcaccatctccagagacaacgccaagaactcactgtatctgcagatgaacagcctgagagccgaggacacggctgtatattactgtgcgagaggagattataattcgggcatctattactttcccggggactactggggccagggcaccctggtcaccgtctcctcg

SEQ ID NO: 58 - protein, 123 aa, Homo sapiens
EVQLVESGGGSVQPGGSLRLSCVASGFIFRNSWMTWVRQDPGKGLEWVANIKEDGSRTYYVDSVKGRFTISRDNAKNSLYLQMNSLRAEDTAVYYCARGDYNSGIYYFPGDYWGQGTLVTVSS

SEQ ID NO: 59 - DNA, 336 bp, Homo sapiens
  V_region 70..117: note = complementarity determining region (CDR) VK-CDR1
  V_region 163..183: note = complementarity determining region (CDR) VK-CDR2
  V_region 280..306: note = complementarity determining region (CDR) VK-CDR3
  source 1..336: mol_type = other DNA
  CDS 1..336: note = NI-302.7A8 VK variable light-kappa chain (VK) sequence
gatgttgtgatgactcagtctccactctccctgcccgtcacccttggacagccggcctccatctcctgtaggtctagtcaaagcctcgtatacagtgatggaaacacctacttgaattggtttcagcagaggccaggccagtctccaaggcgcctcatttataaggtttctaaccgggactctggggtcccagacagattcagcggcagtgggtcaggcactgatttcacactgagaatcagcagggtggaggctgaggatgttggcatttattactgcatgcaaggtacacactggcctgggacgttcggccaagggaccaaggtggagatcaaa

SEQ ID NO: 60 - protein, 112 aa, Homo sapiens
DVVMTQSPLSLPVTLGQPASISCRSSQSLVYSDGNTYLNWFQQRPGQSPRRLIYKVSNRDSGVPDRFSGSGSGTDFTLRISRVEAEDVGIYYCMQGTHWPGTFGQGTKVEIK

SEQ ID NO: 61 - DNA, 381 bp, Homo sapiens
  V_region 91..108: note = complementarity determining region (CDR) VH-CDR1
  V_region 151..198: note = complementarity determining region (CDR) VH-CDR2
  V_region 295..348: note = complementarity determining region (CDR) VH-CDR3
  source 1..381: mol_type = other DNA
  CDS 1..381: note = NI-302.78H12 VH variable heavy chain (VH) sequence
caggtgcagctgcaggagtcgggcccaggactggtgaagccttcggagaccctgtccctcacctgtcttgtctctagttactccatcagcaatggttactactggggctggattcggcagcccccagggaaggggctggagtggattgggagtatctatcataatgggaacacctattacaacccgtccctcaagagtcgagtcatcatttcagtagacacgtccaagaaccagttctccctgaagttgaggtctgtgaccgccgcagacacggccgtgtactactgtgcgatgccaagtgccacctattattatggttcggggactcaattccatgcgtttgatgtctggggccaagggaccacggtcaccgtctcctcg

SEQ ID NO: 62 - protein, 127 aa, Homo sapiens
QVQLQESGPGLVKPSETLSLTCLVSSYSISNGYYWGWIRQPPGKGLEWIGSIYHNGNTYYNPSLKSRVIISVDTSKNQFSLKLRSVTAADTAVYYCAMPSATYYYGSGTQFHAFDVWGQGTTVTVSS

SEQ ID NO: 63 - DNA, 333 bp, Homo sapiens
  V_region 67..108: note = complementarity determining region (CDR) VL-CDR1
  V_region 154..174: note = complementarity determining region (CDR) VL-CDR2
  V_region 271..303: note = complementarity determining region (CDR) VL-CDR3
  source 1..333: mol_type = other DNA
  CDS 1..333: note = NI-302.78H12 VL variable light chain (VL) sequence
cagtctgccctgactcagcctcgctcagtgtccgggtctcctggacagtcagtcaccatctcctgcactggaaccagcagagatgttggtaattataactatgtctcctggtaccaacaacacccaggcgaagtccccaaactcataatttatgatgtcagtgagcggccctcaggggtccctgatcgcttctctggctccaagtctggcaacacggcctcgctgaccatctctgggctccaggctgaggatgaggctgactattactgctgctcatatgctggcagttacaccttcgaggtatttggcggagggaccaagctgaccgtccta

SEQ ID NO: 64 - protein, 111 aa, Homo sapiens
QSALTQPRSVSGSPGQSVTISCTGTSRDVGNYNYVSWYQQHPGEVPKLIIYDVSERPSGVPDRFSGSKSGNTASLTISGLQAEDEADYYCCSYAGSYTFEVFGGGTKLTVL

SEQ ID NO: 65 - DNA, 360 bp, Homo sapiens
  V_region 91..105: note = complementarity determining region (CDR) VH-CDR1
  V_region 148..195: note = complementarity determining region (CDR) VH-CDR2
  V_region 292..327: note = complementarity determining region (CDR) VH-CDR3
  source 1..360: mol_type = other DNA
  CDS 1..360: note = NI-302.71F6 VH variable heavy chain (VH) sequence
caggtgcagctacagcagtggggcgcaggactattgaagccttcggagaccctgtccctcacgtgcgctgtctatggtgggtccctcagtggttactactggagctggatccgccagcccccagggaaggggctggagtggataggggaagtcaatcatagtggaggcaccaacctcaattcgtccctcaagagtcgagtcatcatttcagtagacaagtccaagaagcagttctccctgaaactgagctctgtgaccgccgcggacacggctatgtacttctgtgcgagaggatacagctatgacccaaaatactactttgactcctggagccagggcaccctggtcaccgtctcctcg

SEQ ID NO: 66 - protein, 120 aa, Homo sapiens
QVQLQQWGAGLLKPSETLSLTCAVYGGSLSGYYWSWIRQPPGKGLEWIGEVNHSGGTNLNSSLKSRVIISVDKSKKQFSLKLSSVTAADTAMYFCARGYSYDPKYYFDSWSQGTLVTVSS

SEQ ID NO: 67 - DNA, 330 bp, Homo sapiens
  V_region 67..108: note = complementarity determining region (CDR) VL-CDR1
  V_region 154..174: note = complementarity determining region (CDR) VL-CDR2
  V_region 271..300: note = complementarity determining region (CDR) VL-CDR3
  source 1..330: mol_type = other DNA
  CDS 1..330: note = NI-302.71F6 VL variable light chain (VL) sequence
cagtctgccctgactcagcctgcctccgtgtctgggtctcctggacaggcgatcaccatctcctgcactggaaccagtagtgatattgggagttatgattttgtctcctggtaccagcaggacccaggcaaagcccccaaagtcattatttatggggtcaataagcggccctcaggggtttctaatcgcttctctggctccaagtctggcaacacggcctccctgacaatctctggactccaggctgacgacgaggctgattattactgctgctcatatgctggtagtaccacttgggtgttcggcggagggaccaaactgaccgtccta

SEQ ID NO: 68 - protein, 110 aa, Homo sapiens
QSALTQPASVSGSPGQAITISCTGTSSDIGSYDFVSWYQQDPGKAPKVIIYGVNKRPSGVSNRFSGSKSGNTASLTISGLQADDEADYYCCSYAGSTTWVFGGGTKLTVL

SEQ ID NO: 69 - DNA, 363 bp, Homo sapiens
  V_region 91..105: note = complementarity determining region (CDR) VH-CDR1
  V_region 148..198: note = complementarity determining region (CDR) VH-CDR2
  V_region 295..330: note = complementarity determining region (CDR) VH-CDR3
  source 1..363: mol_type = other DNA
  CDS 1..363: note = NI-302.11H6 VH variable heavy chain (VH) sequence
gaggtgcagctggtgcagtctggagctgtgatgaagaagcctggagactcagtgagggtctcctgcagggcttctacttacagcttttccacctatagtttcacctgggtgcgacaggtccctggacaaggccttgagtggatgggatggatcagcgcttataatggtcacacaaactatgtagacagcttccagggcagactcacgttgaccacagacacatccgcgagtacagcgtacatggaactgaggagcctcagatctgacgacacggccatctattattgtgcggctgtagacaccacttactactattacggcatggacgtctggggccaaggcaccctggtcaccgtctcctcg

SEQ ID NO: 70 - protein, 121 aa, Homo sapiens
EVQLVQSGAVMKKPGDSVRVSCRASTYSFSTYSFTWVRQVPGQGLEWMGWISAYNGHTNYVDSFQGRLTLTTDTSASTAYMELRSLRSDDTAIYYCAAVDTTYYYYGMDVWGQGTLVTVSS

SEQ ID NO: 71 - DNA, 330 bp, Homo sapiens
  V_region 67..108: note = complementarity determining region (CDR) VL-CDR1
  V_region 154..174: note = complementarity determining region (CDR) VL-CDR2
  V_region 271..300: note = complementarity determining region (CDR) VL-CDR3
  source 1..330: mol_type = other DNA
  CDS 1..330: note = NI-302.11H6 VL variable light chain (VL) sequence
cagactgtggtgactcaggagccaacgttctcagtgtcccctggagggacagtcacactcacttgtgccttgaggtttggctcagtctctagtagctactatcccagctggttccagcagaccccaggccaggctccacgcacgctcatctacagcacaaacacccgctcttcgggggtccctgctcgattctctggctccattcttgggaacaaagctgccctcaccatcgcgggggcccaggcaaatgatgaggctgactattactgtgtgctgtatatgggtagtggaatcggggtgttcggcggagggaccaagttgaccgtccta

SEQ ID NO: 72 - protein, 110 aa, Homo sapiens
QTVVTQEPTFSVSPGGTVTLTCALRFGSVSSSYYPSWFQQTPGQAPRTLIYSTNTRSSGVPARFSGSILGNKAALTIAGAQANDEADYYCVLYMGSGIGVFGGGTKLTVL

SEQ ID NO: 73 - DNA, 357 bp, Homo sapiens
  V_region 88..105: note = complementarity determining region (CDR) VH-CDR1
  V_region 148..198: note = complementarity determining region (CDR) VH-CDR2
  V_region 295..324: note = complementarity determining region (CDR) VH-CDR3
  source 1..357: mol_type = other DNA
  CDS 1..357: note = NI-302.3D8 VH variable heavy chain (VH) sequence
gaggtgcagctggtgcagtctgggggaggcttggtacagcctggggggtccctgagactctcttgtgaagcctccggattcatctttaaaacctatgccatgagctgggtccgccagcttcccgggagggggctggaatgggtctcagctataagtgccactggtggaagcaccttctacgcagagtccgtgaagggccggctcaccatttccagagacactgccaagaatacagtgtatctgcaaatgaacaacctgagagccgaagacacggccatgtattactgtgcgaaagggtcgactgcggtatatctctttgactcctggggccagggaaccctggtcaccgtctcctcg

SEQ ID NO: 74 - protein, 119 aa, Homo sapiens
EVQLVQSGGGLVQPGGSLRLSCEASGFIFKTYAMSWVRQLPGRGLEWVSAISATGGSTFYAESVKGRLTISRDTAKNTVYLQMNNLRAEDTAMYYCAKGSTAVYLFDSWGQGTLVTVSS

SEQ ID NO: 75 - DNA, 321 bp, Homo sapiens
  V_region 70..102: note = complementarity determining region (CDR) VK-CDR1
  V_region 148..168: note = complementarity determining region (CDR) VK-CDR2
  V_region 265..291: note = complementarity determining region (CDR) VK-CDR3
  source 1..321: mol_type = other DNA
  CDS 1..321: note = NI-302.3D8 VK variable light-kappa chain (VK) sequence
gacatccagatgacccagtctccgtcctcactgtctgcatctgtaggggacagagtcaccctcacttgtcgggcgagtcaggacatcagaaatttcttggcctggattcagcagaagccagggaaaccccctaagtccctgatctatgctgcgtccactttgcaaagtggggtcccatcacgattcagcggcagtggatccgggacagatttcactctcaccatcagcagcctgcaccctgaagattttgctacttattactgccagcagttttataattaccctccgacgttcggccaagggaccaaggtggagatcaaa

SEQ ID NO: 76 - protein, 107 aa, Homo sapiens
DIQMTQSPSSLSASVGDRVTLTCRASQDIRNFLAWIQQKPGKPPKSLIYAASTLQSGVPSRFSGSGSGTDFTLTISSLHPEDFATYYCQQFYNYPPTFGQGTKVEIK

SEQ ID NO: 77 - DNA, 360 bp, Homo sapiens
  V_region 91..105: note = complementarity determining region (CDR) VH-CDR1
  V_region 154..201: note = complementarity determining region (CDR) VH-CDR2
  V_region 298..327: note = complementarity determining region (CDR) VH-CDR3
  source 1..360: mol_type = other DNA
  CDS 1..360: note = NI-302.18A1 VH variable heavy chain (VH) sequence
cagctgcagctgcaggagtcgggcccaggactagtgaagccttcggaggccctgtccctcacctgcactgtctctggtggctccatcactactgattattactattggggctggatccgccagtccccaggcaagggactagagtgggttgggacaatatactttggtggggccacctactacaatccgtccctcaggaaccgggtctcgatatctgtggacacgtccaacactcgcctctccctgagacttatctctctgagcgccgctgacacggccgtctattattgtgcgagagtgggctacttggataggagtggtcttcttgtgggccagggcaccctggtcaccgtctcctcg

SEQ ID NO: 78 - protein, 120 aa, Homo sapiens
QLQLQESGPGLVKPSEALSLTCTVSGGSITTDYYYWGWIRQSPGKGLEWVGTIYFGGATYYNPSLRNRVSISVDTSNTRLSLRLISLSAADTAVYYCARVGYLDRSGLLVGQGTLVTVSS

SEQ ID NO: 79 - DNA, 336 bp, Homo sapiens
  V_region 70..117: note = complementarity determining region (CDR) VK-CDR1
  V_region 163..183: note = complementarity determining region (CDR) VK-CDR2
  V_region 280..306: note = complementarity determining region (CDR) VK-CDR3
  source 1..336: mol_type = other DNA
  CDS 1..336: note = NI-302.18A1 VK variable light-kappa chain (VK) sequence
gaaattgtgctgacgcagtctccactctccgtgcccgtcacccccggagagccggcctccatctcctgcaggtctagtcagagcctcctgcataataatggatacaactatttggattggtacctgaagaagcctgggcagtctccacaactcctgatctatttgggctctactcgggcctccggggtccctgacaggttcagtgccagtggatcaggcacagactttacactggaaatcagcagagtggaggctgaagatgttggcgtttactactgcatgcaagctctgcagactcctccgactttcggcagagggaccaaggtggagatcaaa

SEQ ID NO: 80 - protein, 112 aa, Homo sapiens
EIVLTQSPLSVPVTPGEPASISCRSSQSLLHNNGYNYLDWYLKKPGQSPQLLIYLGSTRASGVPDRFSASGSGTDFTLEISRVEAEDVGVYYCMQALQTPPTFGRGTKVEIK

SEQ ID NO: 81 - DNA, 366 bp, Homo sapiens
  V_region 91..105: note = complementarity determining region (CDR) VH-CDR1
  V_region 148..204: note = complementarity determining region (CDR) VH-CDR2
  V_region 301..333: note = complementarity determining region (CDR) VH-CDR3
  source 1..366: mol_type = other DNA
  CDS 1..366: note = NI-302.8F1 VH variable heavy chain (VH) sequence
gaggtgcagctggtggagtctgggggaggcttggtgaagccgggggggtcccttacaatctcctgtgcagcctctggtttcaccttcagtaatgcctggatgaactgggtccgccaggctccaggtaaggggctggagtgggtcggccatattagaacgcaagctgaaggagggacatcagactatgctgcacccgtgaaaggcagattcaccatctcaagagatgactcaaaaaacacgctgtatctgcaaatgaacagcctgaaaaccgaggacacagccgtatattattgtatcccccccccctactactactattacggtctggacgtctggggccaagggaccacggtcaccgtctcctcg

SEQ ID NO: 82 - protein, 122 aa, Homo sapiens
EVQLVESGGGLVKPGGSLTISCAASGFTFSNAWMNWVRQAPGKGLEWVGHIRTQAEGGTSDYAAPVKGRFTISRDDSKNTLYLQMNSLKTEDTAVYYCIPPPYYYYYGLDVWGQGTTVTVSS

SEQ ID NO: 83 - DNA, 327 bp, Homo sapiens
  V_region 67..108: note = complementarity determining region (CDR) VL-CDR1
  V_region 154..174: note = complementarity determining region (CDR) VL-CDR2
  V_region 271..297: note = complementarity determining region (CDR) VL-CDR3
  source 1..327: mol_type = other DNA
  CDS 1..327: note = NI-302.8F1 VL variable light chain (VL) sequence
cagtctgccctgactcagcctgcctccgtgtctgggtctcctggacagtcgatcaccatctcctgcactggagccagcagtgatgttgggacttatgaccttgtctcctggtaccaacaacatccaggcaaagcccccaaactcattatttatgaggtcaataagcggccctcaggggtttcttatcgcttctctgcctccaagtctgccaacacggcctccctgacaatatctgggctccaggctgaggacgaggctgaatattactgctgctcatatgcaggttatagcacggtattcggcggagggaccaagctgaccgtccta

SEQ ID NO: 84 - protein, 109 aa, Homo sapiens
QSALTQPASVSGSPGQSITISCTGASSDVGTYDLVSWYQQHPGKAPKLIIYEVNKRPSGVSYRFSASKSANTASLTISGLQAEDEAEYYCCSYAGYSTVFGGGTKLTVL

SEQ ID NO: 85 - DNA, 357 bp, Homo sapiens
  V_region 91..105: note = complementarity determining region (CDR) VH-CDR1
  V_region 148..195: note = complementarity determining region (CDR) VH-CDR2
  V_region 292..324: note = complementarity determining region (CDR) VH-CDR3
  source 1..357: mol_type = other DNA
  CDS 1..357: note = NI-302.52C9 VH variable heavy chain (VH) sequence
gaggtgcagctggtgcagtctgggggaggcttggtccaacctggggggtccctgagactctcctgtgcaggctctggattcaccgtcagtgacacctacatgagttgggtccgccaggctccagggaaggggctggagtgggtctcaggtattcatgccggtggtgaaacatattacgcagactccgtgaagggccgattcaccatctccagagacaactccaagaacacgctgtatcttcaaatgaataggctgacacctgaggacacggctgtcttttattgtgcgagacactactacggtaatgacgacgacactgattattggggccagggaaccctggtcaccgtctcctcg

SEQ ID NO: 86 - protein, 119 aa, Homo sapiens
EVQLVQSGGGLVQPGGSLRLSCAGSGFTVSDTYMSWVRQAPGKGLEWVSGIHAGGETYYADSVKGRFTISRDNSKNTLYLQMNRLTPEDTAVFYCARHYYGNDDDTDYWGQGTLVTVSS

SEQ ID NO: 87 - DNA, 336 bp, Homo sapiens
  V_region 70..117: note = complementarity determining region (CDR) VK-CDR1
  V_region 163..183: note = complementarity determining region (CDR) VK-CDR2
  V_region 280..306: note = complementarity determining region (CDR) VK-CDR3
  source 1..336: mol_type = other DNA
  CDS 1..336: note = NI-302.52C9 VK variable light-kappa chain (VK) sequence
gatgttgtgatgactcagtctccactctccctgcccgtcacccctggagagccggcctccatctcctgcaggtctagtcagagcctcctgcatagtaatggatacaactatttggattggtacgtgcagaagccagggcagtctccacagctcctcatctatttgggttctactcgggcctccggggtccctgacagattcagtggcagtggatcaggcacagattttacactgaaaatcagcagagtggaggctgaggatgttggggtttattactgcttacaagctcaacaaattccgtggacgttcggccaagggaccaaggtggagatcaaa

SEQ ID NO: 88 - protein, 112 aa, Homo sapiens
DVVMTQSPLSLPVTPGEPASISCRSSQSLLHSNGYNYLDWYVQKPGQSPQLLIYLGSTRASGVPDRFSGSGSGTDFTLKISRVEAEDVGVYYCLQAQQIPWTFGQGTKVEIK

SEQ ID NO: 89 - DNA, 369 bp, Homo sapiens
  V_region 91..105: note = complementarity determining region (CDR) VH-CDR1
  V_region 154..201: note = complementarity determining region (CDR) VH-CDR2
  V_region 298..336: note = complementarity determining region (CDR) VH-CDR3
  source 1..369: mol_type = other DNA
  CDS 1..369: note = NI-302.46C9 VH variable heavy chain (VH) sequence
caggtgcagctgcaggagtcgggcccaggactggtaaagccttcacagaccctgtccctcacctgcactgtttctggtgcctccgtcagcagtggtgcctactactggagttggatccggcagcccgccgggaagcgactggagtggattgggcgtgtctatcccacttggagcaccaactacaacccctccctcgagagtcgagtcaccatatcgttagacacgtccaacaaccagttctccctgaagctgacctctttgactgccgcagacacggccgtttattactgtgcgagagaggctcctggtgactacgatgctgcgcccctagcctactggggccagggcaccctggtcaccgtctcctcg

SEQ ID NO: 90 - protein, 123 aa, Homo sapiens
QVQLQESGPGLVKPSQTLSLTCTVSGASVSSGAYYWSWIRQPAGKRLEWIGRVYPTWSTNYNPSLESRVTISLDTSNNQFSLKLTSLTAADTAVYYCAREAPGDYDAAPLAYWGQGTLVTVSS

SEQ ID NO: 91 - DNA, 321 bp, Homo sapiens
  V_region 70..102: note = complementarity determining region (CDR) VK-CDR1
  V_region 148..168: note = complementarity determining region (CDR) VK-CDR2
  V_region 265..291: note = complementarity determining region (CDR) VK-CDR3
  source 1..321: mol_type = other DNA
  CDS 1..321: note = NI-302.46C9 VK variable light-kappa chain (VK) sequence
gacatccagatgacccagtctccatcctccctgtctgcatctgttggagacagagtcaccatcacttgccgggcaagtcagtacattagccactatttaaattggtatcggcagaaaccagggaaagcccctcagctcgtaatctatgctgcatccagtttgcaaagtgaggtcccatcaaggttcagtgggagtggatctgggccagagttcactctcaccatcagcagtctgcaacctgaagattttgcaacttattactgtcaacagagttacactacccctcgaacttttggccaggggaccaagctggagatcaaa

SEQ ID NO: 92 - protein, 107 aa, Homo sapiens
DIQMTQSPSSLSASVGDRVTITCRASQYISHYLNWYRQKPGKAPQLVIYAASSLQSEVPSRFSGSGSGPEFTLTISSLQPEDFATYYCQQSYTTPRTFGQGTKLEIK

SEQ ID NO: 93 - protein, 19 aa, synthetic construct
  REGION 1..19: note = BSA-coupled synthetic peptides (Schafer-N, Denmark) of the HTT exon 1 N-terminal amino acids 1-19
MATLEKLMKAFESLKSFQQ

SEQ ID NO: 94 - protein, 21 aa, synthetic construct
  REGION 1..21: note = BSA-coupled synthetic peptides (Schafer-N, Denmark) of the HTT exon 1 P-rich domain
PPQLPQPPPQAQPLLPQPQPP

SEQ ID NO: 95 - protein, 11 aa, synthetic construct
  REGION 1..11: note = BSA-coupled synthetic peptides (Schafer-N, Denmark) of the HTT exon 1polyP repeat
PPPPPPPPPPP

SEQ ID NO: 96 - protein, 14 aa, synthetic construct
  REGION 1..14: note = BSA-coupled synthetic peptides (Schafer-N, Denmark) of the HTT exon 1 C-terminal amino acids
PPGPAVAEEPLHRP

SEQ ID NO: 97 - DNA, 369 bp, Homo sapiens
  V_region 91..105: note = complementarity determining region (CDR) VH-CDR1
  V_region 148..198: note = complementarity determining region (CDR) VH-CDR2
  V_region 295..336: note = complementarity determining region (CDR) VH-CDR3
  source 1..369: mol_type = other DNA
  CDS 1..369: note = NI-302.33C11-PIMC VH variable heavy chain (VH) sequence
caggtgcagctggtggagtctgggggaggcgttgtccagcctgggaactccctgagactctcctgtgcagcgtctggattcaggttcagtgactttggcatgcactgggtccgccaggctccaggcaagggactggagtggctggcacttatatggtatgatggagggtataagtactatgcagactccgtgaagggccgattcaccatctccagagacaattccaagaatacgatgtttctacaaatgaacagcctgagagccgaggacacggctgtttattactgtgcgacccacctagaatattgcagtagaaccacctgctatctcggccactggggccagggaaccctggtcaccgtctcctcg

SEQ ID NO: 98 - protein, 123 aa, Homo sapiens
QVQLVESGGGVVQPGNSLRLSCAASGFRFSDFGMHWVRQAPGKGLEWLALIWYDGGYKYYADSVKGRFTISRDNSKNTMFLQMNSLRAEDTAVYYCATHLEYCSRTTCYLGHWGQGTLVTVSS

SEQ ID NO: 99 - DNA, 321 bp, Homo sapiens
  V_region 70..102: note = complementarity determining region (CDR) VK-CDR1
  V_region 148..168: note = complementarity determining region (CDR) VK-CDR2
  V_region 265..291: note = complementarity determining region (CDR) VK-CDR3
  source 1..321: mol_type = other DNA
  CDS 1..321: note = NI-302.33C11-PIMC VK variable kappa-light chain (VK) sequence
gacatccagttgacccagtctccgtccttcctatctgcgtctgtgggagacacagtcaccttcacttgccgggccagtcagggcattagcgattatttagcctggtttcagcagaaaccagggattgcccctaagctcctgatctatgctgcgtccactttgcaaaccggggtcccatcaaggttcagcggcagtggatctgggacagaattcactctcacaatccgcagcctgcagtctgaagattttggaacttattactgtcagcagcttaaaacttacccgtacacttttggccaggggaccaagctggagatcaaa

SEQ ID NO: 100 - protein, 107 aa, Homo sapiens
DIQLTQSPSFLSASVGDTVTFTCRASQGISDYLAWFQQKPGIAPKLLIYAASTLQTGVPSRFSGSGSGTEFTLTIRSLQSEDFGTYYCQQLKTYPYTFGQGTKLEIK

SEQ ID NO: 101 - DNA, 339 bp, Homo sapiens
  V_region 70..120: note = complementarity determining region (CDR) VK-CDR1
  V_region 166..186: note = complementarity determining region (CDR) VK-CDR2
  V_region 283..309: note = complementarity determining region (CDR) VK-CDR3
  source 1..339: mol_type = other DNA
  CDS 1..339: note = NI-307.63F3-PIMC VK variable kappa-light chain (VK) sequence
gatattgtgatgactcaatcaccagactccctggctgtgtctctgggcgagagggccaccatcaactgcaagtccaatcagagtcttttctacagttccaacaataacaactacttagcttggtaccagcacaaatccggacagcctcctaagctgctcgtttactggggatctacccgggaatccggggtccctgaccgcttcagtggcagcgggtctgggactgacttcactctcaccatcagtagcctgcaggctgaggatgttgcaatttattactgtcaccaatattatcataatccgtacacttttggccaggggaccaagctggagatcaaa

SEQ ID NO: 102 - protein, 113 aa, Homo sapiens
DIVMTQSPDSLAVSLGERATINCKSNQSLFYSSNNNNYLAWYQHKSGQPPKLLVYWGSTRESGVPDRFSGSGSGTDFTLTISSLQAEDVAIYYCHQYYHNPYTFGQGTKLEIK

SEQ ID NO: 103 - DNA, 339 bp, Homo sapiens
  V_region 70..120: note = complementarity determining region (CDR) VK-CDR1
  V_region 166..186: note = complementarity determining region (CDR) VK-CDR2
  V_region 283..309: note = complementarity determining region (CDR) VK-CDR3
  source 1..339: mol_type = other DNA
  CDS 1..339: note = NI-307.63F3-PIMC-NS VK variable kappa-light chain (VK) sequence
gatattgtgatgactcaatcaccagactccctggctgtgtctctgggcgagagggccaccatcaactgcaagtcctcacagagtcttttctacagttccaacaataacaactacttagcttggtaccagcacaaatccggacagcctcctaagctgctcgtttactggggatctacccgggaatccggggtccctgaccgcttcagtggcagcgggtctgggactgacttcactctcaccatcagtagcctgcaggctgaggatgttgcaatttattactgtcaccaatattatcataatccgtacacttttggccaggggaccaagctggagatcaaa

SEQ ID NO: 104 - protein, 113 aa, Homo sapiens
DIVMTQSPDSLAVSLGERATINCKSSQSLFYSSNNNNYLAWYQHKSGQPPKLLVYWGSTRESGVPDRFSGSGSGTDFTLTISSLQAEDVAIYYCHQYYHNPYTFGQGTKLEIK

SEQ ID NO: 105 - DNA, 339 bp, Homo sapiens
  V_region 70..120: note = complementarity determining region (CDR) VK-CDR1
  V_region 166..186: note = complementarity determining region (CDR) VK-CDR2
  V_region 283..309: note = complementarity determining region (CDR) VK-CDR3
  source 1..339: mol_type = other DNA
  CDS 1..339: note = NI-307.63F3-PIMC-SG VK variable kappa-light chain (VK) sequence
gatattgtgatgactcaatcaccagactccctggctgtgtctctgggcgagagggccaccatcaactgcaagtccaatcagggccttttctacagttccaacaataacaactacttagcttggtaccagcacaaatccggacagcctcctaagctgctcgtttactggggatctacccgggaatccggggtccctgaccgcttcagtggcagcgggtctgggactgacttcactctcaccatcagtagcctgcaggctgaggatgttgcaatttattactgtcaccaatattatcataatccgtacacttttggccaggggaccaagctggagatcaaa

SEQ ID NO: 106 - protein, 113 aa, Homo sapiens
DIVMTQSPDSLAVSLGERATINCKSNQGLFYSSNNNNYLAWYQHKSGQPPKLLVYWGSTRESGVPDRFSGSGSGTDFTLTISSLQAEDVAIYYCHQYYHNPYTFGQGTKLEIK

SEQ ID NO: 107 - DNA, 339 bp, Homo sapiens
  V_region 70..120: note = complementarity determining region (CDR) VK-CDR1
  V_region 166..186: note = complementarity determining region (CDR) VK-CDR2
  V_region 283..309: note = complementarity determining region (CDR) VK-CDR3
  source 1..339: mol_type = other DNA
  CDS 1..339: note = NI-307.63F3-PIMC-NQ VK variable kappa-light chain (VK) sequence
gatattgtgatgactcaatcaccagactccctggctgtgtctctgggcgagagggccaccatcaactgcaagtcccaacagagtcttttctacagttccaacaataacaactacttagcttggtaccagcacaaatccggacagcctcctaagctgctcgtttactggggatctacccgggaatccggggtccctgaccgcttcagtggcagcgggtctgggactgacttcactctcaccatcagtagcctgcaggctgaggatgttgcaatttattactgtcaccaatattatcataatccgtacacttttggccaggggaccaagctggagatcaaa

SEQ ID NO: 108 - protein, 113 aa, Homo sapiens
DIVMTQSPDSLAVSLGERATINCKSQQSLFYSSNNNNYLAWYQHKSGQPPKLLVYWGSTRESGVPDRFSGSGSGTDFTLTISSLQAEDVAIYYCHQYYHNPYTFGQGTKLEIK

SEQ ID NO: 109 - DNA, 321 bp, Homo sapiens
  V_region 70..102: note = complementarity determining region (CDR) VK-CDR1
  V_region 148..168: note = complementarity determining region (CDR) VK-CDR2
  V_region 265..291: note = complementarity determining region (CDR) VK-CDR3
  source 1..321: mol_type = other DNA
  CDS 1..321: note = NI-302.35C1-PIMC VK variable kappa-light chain (VK) sequence
gaaattgtgctgactcagtctccagccaccctgtctttgtctccaggggaaagagccaccctctcctgcagggccagtcaaagtgttgacaaccagtttgcctggtaccaacagaaacctggccaggctcccaggctcctcatttatgatgcatccaggagggcccctggcatcccagacaggttcagtggcagtgggtctgggacagacttcactctcaccattagcagcctagagcctgaagatttcgcaatttattactgtcagcatcgttacacctggctctacacttttggccaggggaccaagctggagatcaaa

SEQ ID NO: 110 - protein, 107 aa, Homo sapiens
EIVLTQSPATLSLSPGERATLSCRASQSVDNQFAWYQQKPGQAPRLLIYDASRRAPGIPDRFSGSGSGTDFTLTISSLEPEDFAIYYCQHRYTWLYTFGQGTKLEIK

SEQ ID NO: 111 - DNA, 336 bp, Homo sapiens
  V_region 70..117: note = complementarity determining region (CDR) VK-CDR1
  V_region 163..183: note = complementarity determining region (CDR) VK-CDR2
  V_region 280..306: note = complementarity determining region (CDR) VK-CDR3
  source 1..336: mol_type = other DNA
  CDS 1..336: note = NI-302.31F11-PIMC VK variable kappa-light chain (VK) sequence
gatattgtgatgactcaatcaccactctccctgcccgtcgcccctggagagccggcctccatctcctgcaggtctagtcagagcctcctatacagtaatggatacaactatttggattggtacctgcagaagccagggaagcctccacagctcctggtctatttgggttctgatcgggcctccggggtccctgacaggttcagtggcagtggatcaggcaaagattttacactgaacatcagcagagtggaggctgaggatgttggggtttattactgcatgcaaggtctacaaagtccgtggacgttcggccaagggaccaaggtggaaatcaaa

SEQ ID NO: 112 - protein, 112 aa, Homo sapiens
DIVMTQSPLSLPVAPGEPASISCRSSQSLLYSNGYNYLDWYLQKPGKPPQLLVYLGSDRASGVPDRFSGSGSGKDFTLNISRVEAEDVGVYYCMQGLQSPWTFGQGTKVEIK

SEQ ID NO: 113 - DNA, 345 bp, Homo sapiens
  V_region 70..129: note = complementarity determining region (CDR) VK-CDR1
  V_region 175..195: note = complementarity determining region (CDR) VK-CDR2
  V_region 292..315: note = complementarity determining region (CDR) VK-CDR3
  source 1..345: mol_type = other DNA
  CDS 1..345: note = NI-302.2A2-PIMC VK variable kappa-light chain (VK) sequence
gatattgtgatgactcaatcaccagactccctggctgtgtctctgggcgagagggccaccatcaactgcaagtccagccagagtcttttatacacctccaaaaataaggacagtaagaactacttaggttggtaccagcagaaaccaggacagcctcctaagctgctcatttactgggcatctacccgggaatccggggtccctgaccgattcagtggcagcgggtctgggacagatttcactctcaccatcagcagcctgcaggctgaggatgtggcagtttattactgtcagcagtattatactactcctcagttcggcggagggaccaaggtggaaatcaaa

SEQ ID NO: 114 - protein, 115 aa, Homo sapiens
DIVMTQSPDSLAVSLGERATINCKSSQSLLYTSKNKDSKNYLGWYQQKPGQPPKLLIYWASTRESGVPDRFSGSGSGTDFTLTISSLQAEDVAVYYCQQYYTTPQFGGGTKVEIK

SEQ ID NO: 115 - DNA, 360 bp, Homo sapiens
  V_region 91..105: note = complementarity determining region (CDR) VH-CDR1
  V_region 148..186: note = complementarity determining region (CDR) VH-CDR2
  V_region 295..327: note = complementarity determining region (CDR) VH-CDR3
  source 1..360: mol_type = other DNA
  CDS 1..360: note = NI-302.74C11-PIMC VH variable heavy chain (VH) sequence
caggtgcagctggtgcaatctgggactgaggtgcagaagcctggggcctcagtaaaagtctcctgcaaggcttctggatacagtttcaccggctactttttgcactgggtacgacaggcccctggacaagggcttgagtggatggggtggatcaaccctaacagtggtgacacaaactatgcagagaagtttcggggcagaatcatcatgaccagggacacgtctgtcagcacagcccacatggagttgagcagcctgagatttgacgacacggccctatattactgtacgagagaggcccctgacccgggcgctgagacggacgtctggggccaaggaaccacggtcaccgtctcctcg

SEQ ID NO: 116 - protein, 120 aa, Homo sapiens
QVQLVQSGTEVQKPGASVKVSCKASGYSFTGYFLHWVRQAPGQGLEWMGWINPNSGDTNYAEKFRGRIIMTRDTSVSTAHMELSSLRFDDTALYYCTREAPDPGAETDVWGQGTTVTVSS

SEQ ID NO: 117 - DNA, 321 bp, Homo sapiens
  V_region 67..99: note = complementarity determining region (CDR) VL-CDR1
  V_region 145..165: note = complementarity determining region (CDR) VL-CDR2
  V_region 262..291: note = complementarity determining region (CDR) VL-CDR3
  source 1..321: mol_type = other DNA
  CDS 1..321: note = NI-302.74C11-PIMC VL variable light chain (VL) sequence
tcctatgagctgactcagccaccctcggtgtcagtgtccccaggacagacggccaggatcacctgctctggagatgcagtgccaaagcagtatatttattggtaccagcagaagccaggccaggcccctattctggtgatatataaagacactcagaggccttcagggatccctgagcgattctctggctccaactcagggacaacagtcacgttgaccataactggcgtccaggcagacgacgagggtgactattactgtcaatcagcagacagtagtgctacttgggtgttcggcggagggaccaaattgaccgtccta

SEQ ID NO: 118 - protein, 107 aa, Homo sapiens
SYELTQPPSVSVSPGQTARITCSGDAVPKQYIYWYQQKPGQAPILVIYKDTQRPSGIPERFSGSNSGTTVTLTITGVQADDEGDYYCQSADSSATWVFGGGTKLTVL

SEQ ID NO: 119 - DNA, 357 bp, Homo sapiens
  V_region 91..105: note = complementarity determining region (CDR) VH-CDR1
  V_region 148..195: note = complementarity determining region (CDR) VH-CDR2
  V_region 292..324: note = complementarity determining region (CDR) VH-CDR3
  source 1..357: mol_type = other DNA
  CDS 1..357: note = NI-302.39G12-PIMC VH variable heavy chain (VH) sequence
gaggtgcagctggtggagtctgggggaggcttggtccacccttgggggtccctgagactctcctgtgcagcctctggattcagcgtctctaattacgccataacttgggtccgccgggctccagggaaggggctgcaatatatttcagtaatttatcgtgatggcaggacatactacggagactccgtgaggggccgcttcaccatctctagggacgattccaagaacactctctatcttcaaatgaacagcctgagatttgaggacacggctgtgtattactgtgcgagagcgcacggccaatattactatggtgtggacgtctggggccaaggaaccacggtcaccgtctcctcg

SEQ ID NO: 120 - protein, 119 aa, Homo sapiens
EVQLVESGGGLVHPWGSLRLSCAASGFSVSNYAITWVRRAPGKGLQYISVIYRDGRTYYGDSVRGRFTISRDDSKNTLYLQMNSLRFEDTAVYYCARAHGQYYYGVDVWGQGTTVTVSS

SEQ ID NO: 121 - DNA, 333 bp, Homo sapiens
  V_region 70..117: note = complementarity determining region (CDR) VK-CDR1
  V_region 163..183: note = complementarity determining region (CDR) VK-CDR2
  V_region 280..303: note = complementarity determining region (CDR) VK-CDR3
  source 1..333: mol_type = other DNA
  CDS 1..333: note = NI-302.39G12-PIMC VK variable kappa-light chain (VK) sequence
gacatcgtgatgacccagtctccactctccctgtccgtcagccctggagagccggcctccatctcctgcaggtctagtcagagcctcctacatagtaatggatacaactatttggattggtaccggcagaaaccagggcagtctccacagctcctgatctatttgagttctaatcggccctccggggtccctgataggttcagtgccagtggatcaggcacagagttcacactgcaaatcagcagagtggaggctgaggatgttggggtttattactgcatgcaatctctgcaaacgttcactttcggcggagggaccaaggtggaaatcaaa

SEQ ID NO: 122 - protein, 111 aa, Homo sapiens
DIVMTQSPLSLSVSPGEPASISCRSSQSLLHSNGYNYLDWYRQKPGQSPQLLIYLSSNRPSGVPDRFSASGSGTEFTLQISRVEAEDVGVYYCMQSLQTFTFGGGTKVEIK

SEQ ID NO: 123 - DNA, 321 bp, Homo sapiens
  V_region 70..105: note = complementarity determining region (CDR) VK-CDR1
  V_region 151..171: note = complementarity determining region (CDR) VK-CDR2
  V_region 268..291: note = complementarity determining region (CDR) VK-CDR3
  source 1..321: mol_type = other DNA
  CDS 1..321: note = NI-302.11A4-PIMC VK variable kappa-light chain (VK) sequence
gaaattgtgctgactcagtctccaggcaccctgtctttgtctccaggagaaagagccaccctctcctgcagggccagtcagagtgttagcagcagctacttcgcctggtaccaacaaaaacctggccaggctcccaggctcctcatctatggtacgtcccgcagggccactgccatcccagacaggttcagtggcagtgggtctgggacagacttcactctcaccatcagcagactggagcctgaagattttgcagtgtattactgtcaacagtatggtagctcgtggacgttcggcccagggaccaaggtggaaatcaaa

SEQ ID NO: 124 - protein, 107 aa, Homo sapiens
EIVLTQSPGTLSLSPGERATLSCRASQSVSSSYFAWYQQKPGQAPRLLIYGTSRRATAIPDRFSGSGSGTDFTLTISRLEPEDFAVYYCQQYGSSWTFGPGTKVEIK

SEQ ID NO: 125 - DNA, 333 bp, Homo sapiens
  V_region 70..117: note = complementarity determining region (CDR) VK-CDR1
  V_region 163..183: note = complementarity determining region (CDR) VK-CDR2
  V_region 280..303: note = complementarity determining region (CDR) VK-CDR3
  source 1..333: mol_type = other DNA
  CDS 1..333: note = NI-302.22H9-PIMC VK variable kappa-light chain (VK) sequence
gatattgtgatgactcaatcaccactctccctgtccgtcagccctggagagccggcctccatctcctgcaggtctagtcagagcctcctacatagtaatggatacaactatttggattggtaccggcagaaaccagggcagtctccacaactcctgatctatttgaattctaatcgggcctccggggtccctgataggttcagtggcagtggatcaggcacagagttcacactgacaatcagcagagtggaggctgaggatgttggggtttattactgcatgcaatctctgcaaacgttcactttcggcggagggaccaaggtggaaatcaaa

SEQ ID NO: 126 - protein, 111 aa, Homo sapiens
DIVMTQSPLSLSVSPGEPASISCRSSQSLLHSNGYNYLDWYRQKPGQSPQLLIYLNSNRASGVPDRFSGSGSGTEFTLTISRVEAEDVGVYYCMQSLQTFTFGGGTKVEIK

SEQ ID NO: 127 - DNA, 357 bp, Homo sapiens
  V_region 91..105: note = complementarity determining region (CDR) VH-CDR1
  V_region 148..198: note = complementarity determining region (CDR) VH-CDR2
  V_region 295..324: note = complementarity determining region (CDR) VH-CDR3
  source 1..357: mol_type = other DNA
  CDS 1..357: note = NI-302.44D7-PIMC VH variable heavy chain (VH) sequence
gaggtgcagctggtggagtctgggggaggcttggtacagcctggggggtccctgagactctcctgtgcagcctctggattcacctttagcagctatgccatgagttgggtccgccaggctccagggaaggggctggagtgggtctcaggtattggttatagtgatactagcacatattacgcagactccgtgaagggccgcttcaccgtctccagagacatttccaagaacacgctgtatctgcaaatgaatagcctgagggccgaggacacggccgtatattactgcgcgaaaggtaccagggactattacggtatggacgtctggggccaaggaaccacggtcaccgtctcctcg

SEQ ID NO: 128 - protein, 119 aa, Homo sapiens
EVQLVESGGGLVQPGGSLRLSCAASGFTFSSYAMSWVRQAPGKGLEWVSGIGYSDTSTYYADSVKGRFTVSRDISKNTLYLQMNSLRAEDTAVYYCAKGTRDYYGMDVWGQGTTVTVSS

SEQ ID NO: 129 - DNA, 381 bp, Homo sapiens
  V_region 91..108: note = complementarity determining region (CDR) VH-CDR1
  V_region 151..198: note = complementarity determining region (CDR) VH-CDR2
  V_region 295..348: note = complementarity determining region (CDR) VH-CDR3
  source 1..381: mol_type = other DNA
  CDS 1..381: note = NI-302.78H12-PIMC VH variable heavy chain (VH) sequence
cagctgcagctgcaggagtcgggcccaggactggtgaagccttcggagaccctgtccctcacctgtcttgtctctagttactccatcagcaatggttactactggggctggattcggcagcccccagggaaggggctggagtggattgggagtatctatcataatgggaacacctattacaacccgtccctcaagagtcgagtcatcatttcagtagacacgtccaagaaccagttctccctgaagttgaggtctgtgaccgccgcagacacggccgtgtactactgtgcgatgccaagtgccacctattattatggttcggggactcaattccatgcgtttgatgtctggggccaagggacaatggtcaccgtctcttcg

SEQ ID NO: 130 - protein, 127 aa, Homo sapiens
QLQLQESGPGLVKPSETLSLTCLVSSYSISNGYYWGWIRQPPGKGLEWIGSIYHNGNTYYNPSLKSRVIISVDTSKNQFSLKLRSVTAADTAVYYCAMPSATYYYGSGTQFHAFDVWGQGTMVTVSS

SEQ ID NO: 131 - DNA, 384 bp, Homo sapiens
  V_region 91..105: note = complementarity determining region (CDR) VH-CDR1
  V_region 148..201: note = complementarity determining region (CDR) VH-CDR2
  V_region 298..351: note = complementarity determining region (CDR) VH-CDR3
  source 1..384: mol_type = other DNA
  CDS 1..384: note = NI-302.15E8 VH variable heavy chain (VH) sequence
gaggtgcagctggtggagtctgggggaggcttgatacagccgggggggtccctgagactctcctgtgcagtctctggattcaccgtcagtagttatagcatgaactgggtccgccaggctccagggaaggggctggagtgggtctcatacactagtagtagcagaagtaataccaaaaagtacgcagactctgtgaagggccgattcaccatctctagagacaatgccaggaactcactctatctgcaaatgaacagcctgagagacgaggacacggctgtgtattactgtgcgagagcaggggacttcggggagttactcactggtgaggggtattacggtatggacgtctggggccaagggaccacggtcaccgtctcctcg

SEQ ID NO: 132 - protein, 128 aa, Homo sapiens
EVQLVESGGGLIQPGGSLRLSCAVSGFTVSSYSMNWVRQAPGKGLEWVSYTSSSRSNTKKYADSVKGRFTISRDNARNSLYLQMNSLRDEDTAVYYCARAGDFGELLTGEGYYGMDVWGQGTTVTVSS

SEQ ID NO: 133 - DNA, 318 bp, Homo sapiens
  V_region 67..99: note = complementarity determining region (CDR) VL-CDR1
  V_region 145..165: note = complementarity determining region (CDR) VL-CDR2
  V_region 262..288: note = complementarity determining region (CDR) VL-CDR3
  source 1..318: mol_type = other DNA
  CDS 1..318: note = NI-302.15E8 VL variable light chain (VL) sequence
tcctatgagctgactcagccaccctcagtgtccgtgtccccaggacagacagccaccatcacctgctcgggagatgaattgggggataaatatgttggttggtatcaacagaagccaggccagtcccctctgctggtcatctatcaagatgcgaagcggccctcagggatccctgagcgattctctggctccaactctgggaacacagccactctgaccatcagcgggacccaggctatggatgaggctgactactactgtcaggcgtgggacagcggcacgatggttttcggcggagggaccaggctgaccgtccta

SEQ ID NO: 134 - protein, 106 aa, Homo sapiens
SYELTQPPSVSVSPGQTATITCSGDELGDKYVGWYQQKPGQSPLLVIYQDAKRPSGIPERFSGSNSGNTATLTISGTQAMDEADYYCQAWDSGTMVFGGGTRLTVL

SEQ ID NO: 135 - DNA, 372 bp, Homo sapiens
  V_region 91..105: note = complementarity determining region (CDR) VH-CDR1
  V_region 148..198: note = complementarity determining region (CDR) VH-CDR2
  V_region 295..339: note = complementarity determining region (CDR) VH-CDR3
  source 1..372: mol_type = other DNA
  CDS 1..372: note = NI-302.15D3 variable heavy chain (VH) sequence
gaggtgcagctggtggagtctgggggagacttagttcagcctggggggtccctaagactctcctgtgcagcctctggattcaccttcagtagctactggatgcactgggtccgccaagctccagggaagggtctggtgtgggtctcacgtattagtaatgatggcagtagcaaaacctacgcggactccgtgaagggccgattcaccatctccagagacaacgccaaaaacacgctgtatctgcaaatgaacagtctgagagccgaggacacggctgtgtattactgtgcaatacttggcggatattgtagtagtaccagttgtcgtccctttgacaactggggccagggaaccctggtcaccgtctcctcg

SEQ ID NO: 136 - protein, 124 aa, Homo sapiens
EVQLVESGGDLVQPGGSLRLSCAASGFTFSSYWMHWVRQAPGKGLVWVSRISNDGSSKTYADSVKGRFTISRDNAKNTLYLQMNSLRAEDTAVYYCAILGGYCSSTSCRPFDNWGQGTLVTVSS

SEQ ID NO: 137 - DNA, 330 bp, Homo sapiens
  V_region 67..108: note = complementarity determining region (CDR) VL-CDR1
  V_region 154..174: note = complementarity determining region (CDR) VL-CDR2
  V_region 271..300: note = complementarity determining region (CDR) VL-CDR3
  source 1..330: mol_type = other DNA
  CDS 1..330: note = NI-302.15D3 VL variable light chain (VL) sequence
cagtctgccctgactcagcctgcctccgtgtctgggtctcctggacagtcgatcaccatctcctgcactggaaccagcagtgacgttggtgtttataactatgtctcctggtaccaacaacacccaggcaaagcccccaaactcatgatttttgatgtcagtaatcggccctcagggatttctaatcgcttctctggctccaagtctggcaacacggcctccctgaccatctctgggctccaggctgaggacgaggctgattattactgcagctcatatacaagcagcgacacttgggtgttcggcggagggaccaagctgaccatccta

SEQ ID NO: 138 - protein, 110 aa, Homo sapiens
QSALTQPASVSGSPGQSITISCTGTSSDVGVYNYVSWYQQHPGKAPKLMIFDVSNRPSGISNRFSGSKSGNTASLTISGLQAEDEADYYCSSYTSSDTWVFGGGTKLTIL

SEQ ID NO: 139 - protein, 8 aa, synthetic construct
  REGION 1..8: note = Epitope of NI-302.33C11 antibody
PPPPPPPP

SEQ ID NO: 140 - protein, 10 aa, synthetic construct
  REGION 1..10: note = Epitope of NI-302.63F3 antibody
PQPPPQAQPL

SEQ ID NO: 141 - protein, 10 aa, synthetic construct
  REGION 1..10: note = Epitope of NI-302.31F11 antibody
PPPQLPQPPP

SEQ ID NO: 142 - protein, 15 aa, synthetic construct
  REGION 1..15: note = Epitope of NI-302.2A2 antibody
QAQPLLPQPQPPPPP

SEQ ID NO: 143 - protein, 15 aa, synthetic construct
  REGION 1..15: note = Epitope of NI302.15D3 antibody
PPPQLPQPPPQAQPL

SEQ ID NO: 144 - protein, 11 aa, synthetic construct
  REGION 1..11: note = Epitope of NI302.15E8 antibody
KAFESLKSFQQ

SEQ ID NO: 145 - protein, 14 aa, synthetic construct
  REGION 1..14: note = Epitope of NI-302.35C1 antibody
PPGPAVAEEPLHRP

SEQ ID NO: 146 - protein, 11 aa, synthetic construct
  REGION 1..11: note = Epitope of NI-302.74C11 antibody
PPPPPPPPPPP

SEQ ID NO: 147 - protein, 11 aa, synthetic construct
  REGION 1..11: note = Epitope of NI-302.15F9 antibody
PPPPPPPPPPP

SEQ ID NO: 148 - protein, 11 aa, synthetic construct
  REGION 1..11: note = Epitope of NI-302.39G12 antibody
PPPPPPPPPPP

SEQ ID NO: 149 - protein, 11 aa, synthetic construct
  REGION 1..11: note = Epitope of NI-302.11A4 antibody
PPPPPPPPPPP

SEQ ID NO: 150 - protein, 11 aa, synthetic construct
  REGION 1..11: note = Epitope of NI-302.22H9 antibody
PPPPPPPPPPP

SEQ ID NO: 151 - protein, 8 aa, synthetic construct
  REGION 1..8: note = Epitope of NI-302.44D7 antibody
PPPPPPPP

SEQ ID NO: 152 - protein, 11 aa, synthetic construct
  REGION 1..11: note = Epitope of NI-302.37C12 antibody
PPPPPPPPPPP

SEQ ID NO: 153 - protein, 11 aa, synthetic construct
  REGION 1..11: note = Epitope of NI-302.55D8 antibody
PPPPPPPPPPP

SEQ ID NO: 154 - protein, 8 aa, synthetic construct
  REGION 1..8: note = Epitope of NI-302.7A8 antibody
PPPPPPPP

SEQ ID NO: 155 - protein, 11 aa, synthetic construct
  REGION 1..11: note = Epitope of NI-302.78H12 antibody
PPPPPPPPPPP

SEQ ID NO: 156 - protein, 11 aa, synthetic construct
  REGION 1..11: note = Epitope of NI-302.71F6 antibody
PPPPPPPPPPP

SEQ ID NO: 157 - protein, 6 aa, synthetic construct
  REGION 1..6: note = Epitope of NI-302.11H6 antibody
PPPPPP

SEQ ID NO: 158 - protein, 8 aa, synthetic construct
  REGION 1..8: note = Epitope of NI-302.3D8 antibody
PPPPPPPP

SEQ ID NO: 159 - protein, 6 aa, synthetic construct
  REGION 1..6: note = Epitope of NI-302.18A1antibody
PPPPPP

SEQ ID NO: 160 - protein, 6 aa, synthetic construct
  REGION 1..6: note = Epitope of NI-302.52C9 antibody
PPPPPP

SEQ ID NO: 161 - protein, 8 aa, synthetic construct
  REGION 1..8: note = Epitope of NI-302.46C9 antibody
PPPPPPPP

SEQ ID NO: 162 - protein, 15 aa, synthetic construct
  REGION 1..15: note = Alternative epitope of NI-302.63F3 antibody
PPPQLPQPPPQAQPL

SEQ ID NO: 163 - protein, 11 aa, synthetic construct
  REGION 1..11: note = Alternative epitope of NI-302.33C11 antibody
PPPPPPPPPPP

SEQ ID NO: 164 - DNA, 366 bp, Homo sapiens
  V_region 91..105: note = complementarity determining region (CDR) VH-CDR1
  V_region 148..204: note = complementarity determining region (CDR) VH-CDR2
  V_region 301..355: note = complementarity determining region (CDR) VH-CDR2
  source 1..366: mol_type = other DNA
  CDS 1..366: note = NI-302.64E5-VH variable heavy chain (VH) sequence
gaggtgcagctggtggagactgggggaggcttggtaaagcctggggggtcccttagactctcctgtgcagcctctggattcactttcgaccaggcctggatgagctgggtccgccaggttccagggaaggggctggagtgggttggccggattaaaacgaaaactgagggtgaagcaacagactacgcagcgcccgtgagaggcagattcaccatctcaagagatgattcagaagacacggtgtttctgcaaatgaacagcctgaaaaccgaggacacagccctgtattactgtacgtcaacgggagtcttagcagcagctgtcgatgtctactggggccagggaaccctggtcaccgtctcctcg

SEQ ID NO: 165 - protein, 122 aa, Homo sapiens
EVQLVETGGGLVKPGGSLRLSCAASGFTFDQAWMSWVRQVPGKGLEWVGRIKTKTEGEATDYAAPVRGRFTISRDDSEDTVFLQMNSLKTEDTALYYCTSTGVLAAAVDVYWGQGTLVTVSS

SEQ ID NO: 166 - DNA, 366 bp, Homo sapiens
  V_region 91..105: note = complementarity determining region (CDR) VH-CDR1
  V_region 148..204: note = complementarity determining region (CDR) VH-CDR2
  V_region 301..355: note = complementarity determining region (CDR) VH-CDR3
  source 1..366: mol_type = other DNA
  CDS 1..366: note = NI-302.64E5-PIMC VH variable heavy chain (VH) sequence
gaggtgcagctggtggagtctgggggaggcttggtaaagcctggggggtcccttagactctcctgtgcagcctctggattcactttcgaccaggcctggatgagctgggtccgccaggttccagggaaggggctggagtgggttggccggattaaaacgaaaactgagggtgaagcaacagactacgcagcgcccgtgagaggcagattcaccatctcaagagatgattcagaagacacggtgtttctgcaaatgaacagcctgaaaaccgaggacacagccctgtattactgtacgtcaacgggagtcttagcagcagctgtcgatgtctactggggccagggcaccctggtcaccgtctcctcg

SEQ ID NO: 167 - protein, 122 aa, Homo sapiens
EVQLVESGGGLVKPGGSLRLSCAASGFTFDQAWMSWVRQVPGKGLEWVGRIKTKTEGEATDYAAPVRGRFTISRDDSEDTVFLQMNSLKTEDTALYYCTSTGVLAAAVDVYWGQGTLVTVSS

SEQ ID NO: 168 - DNA, 339 bp, Homo sapiens
  V_region 70..120: note = complementarity determining region (CDR) VK-CDR1
  V_region 166..186: note = complementarity determining region (CDR) VK-CDR2
  V_region 283..309: note = complementarity determining region (CDR) VK-CDR3
  source 1..339: mol_type = other DNA
  CDS 1..339: note = NI-302.64E5 VK variable light-kappa chain (VK) sequence
gacatccagttgacccagtctccagactccctggctgtgtctctgggcgagagggccaccatgacctgcaagtccagccagagtcttttctacagttacaacaatgagaactacttagcctggtatcagcagagaccaggacagcctcctaagttgctcatttactgggcatctacccgggaatccggggtccctgaccgattcagtggcagcgggtctgggacagatttcactctcaccatcagcagcctgcaggctgaagatgtggcagtttattactgtcagcaatattatagtactcctcagacgttcggccaagggaccaaagtggatatcaaa

SEQ ID NO: 169 - protein, 113 aa, Homo sapiens
DIQLTQSPDSLAVSLGERATMTCKSSQSLFYSYNNENYLAWYQQRPGQPPKLLIYWASTRESGVPDRFSGSGSGTDFTLTISSLQAEDVAVYYCQQYYSTPQTFGQGTKVDIK

SEQ ID NO: 170 - DNA, 339 bp, Homo sapiens
  V_region 70..120: note = complementarity determining region (CDR) VK-CDR1
  V_region 166..186: note = complementarity determining region (CDR) VK-CDR2
  V_region 283..309: note = complementarity determining region (CDR) VK-CDR3
  source 1..339: mol_type = other DNA
  CDS 1..339: note = NI-302.64E5-PIMC VK variable kappa-light chain (VK) sequence
gatattgtgatgactcaatcaccagactccctggctgtgtctctgggcgagagggccaccatgacctgcaagtccagccagagtcttttctacagttacaacaatgagaactacttagcctggtatcagcagagaccaggacagcctcctaagttgctcatttactgggcatctacccgggaatccggggtccctgaccgattcagtggcagcgggtctgggacagatttcactctcaccatcagcagcctgcaggctgaagatgtggcagtttattactgtcagcaatattatagtactcctcagacgttcggccaagggaccaaggtggaaatcaaa

SEQ ID NO: 171 - protein, 113 aa, Homo sapiens
DIVMTQSPDSLAVSLGERATMTCKSSQSLFYSYNNENYLAWYQQRPGQPPKLLIYWASTRESGVPDRFSGSGSGTDFTLTISSLQAEDVAVYYCQQYYSTPQTFGQGTKVEIK

SEQ ID NO: 172 - DNA, 357 bp, Homo sapiens
  V_region 91..105: note = complementarity determining region (CDR) VH-CDR1
  V_region 148..198: note = complementarity determining region (CDR) VH-CDR2
  V_region 295..324: note = complementarity determining region (CDR) VH-CDR3
  source 1..357: mol_type = other DNA
  CDS 1..357: note = NI-302.7D8-VH variable heavy chain (VH) sequence
caggtgcagctggtgcaatctggatctgagttgaagaagcctggggcctcagtgaaggtttcctgcaaggcttctggatacaacttcaataactatgccatcaattggttgcgacaggcccctggacaagggcttgagtggatgggatggatcaacaccatcactgggcacccaacgtatgcccagggcttcaaaggacgatttgtcttctccttggacacctctgtcagcacggcatatctgcagatcagcagcctaaagcctgaggacactgccgtctattactgtgcgagaacttacagtaactacggcgaatttgactactggggccagggaaccctggtcaccgtctcctcg

SEQ ID NO: 173 - protein, 119 aa, Homo sapiens
QVQLVQSGSELKKPGASVKVSCKASGYNFNNYAINWLRQAPGQGLEWMGWINTITGHPTYAQGFKGRFVFSLDTSVSTAYLQISSLKPEDTAVYYCARTYSNYGEFDYWGQGTLVTVSS

SEQ ID NO: 174 - DNA, 333 bp, Homo sapiens
  V_region 67..108: note = complementarity determining region (CDR) VL-CDR1
  V_region 154..174: note = complementarity determining region (CDR) VL-CDR2
  V_region 271..303: note = complementarity determining region (CDR) VL-CDR3
  source 1..333: mol_type = other DNA
  CDS 1..333: note = NI-302.7D8 VL variable light-lambda chain (VL) sequence
cagtctgccctgactcagcctgcctccgtgtctgggtctcgtggacagtcgatcaccatctcctgcactggaaccagcagtgatgttggaagttataaccttgtctcctggtaccaacagtacccaggcaaggcccccaagctcataattcatgagggcagtgagcggccctcaggggtttctaatcgcttctctggctccaagtctggcaacacggcctccctgacaatttctgggctccaggctgaggacgaggctgattattactgctgctcatatgcaggtactactactttcgtgctattcggcggagggaccaagctgaccgtcctc

SEQ ID NO: 175 - protein, 111 aa, Homo sapiens
QSALTQPASVSGSRGQSITISCTGTSSDVGSYNLVSWYQQYPGKAPKLIIHEGSERPSGVSNRFSGSKSGNTASLTISGLQAEDEADYYCCSYAGTTTFVLFGGGTKLTVL

SEQ ID NO: 176 - DNA, 357 bp, Homo sapiens
  V_region 91..105: note = complementarity determining region (CDR) VH-CDR1
  V_region 148..198: note = complementarity determining region (CDR) VH-CDR2
  V_region 295..324: note = complementarity determining region (CDR) VH-CDR2
  source 1..357: mol_type = other DNA
  CDS 1..357: note = NI-302.72F10-VH variable heavy chain (VH) sequence
gaggtgcagctggtggagactgggggaggcttcgtacagcctggggggtccctgagactctcctgtgcagcctctggattcaacttcggcagttatgccatgagctgggtccgccaggctccagggaagggactggagtgggtgtcagatatcagtggtattggtagtaacacatactacgcagactccgtgaagggccgtttcaccatttccagagacaattccgacaatacgttgtacctggacatgagcagcctgagagccgaggacacggccagatattactgtgcgaaggatcgaaagcgcagtggctggtacgaacagtggggccagggcaccctggtcaccgtctcctcg

SEQ ID NO: 177 - protein, 119 aa, Homo sapiens
EVQLVETGGGFVQPGGSLRLSCAASGFNFGSYAMSWVRQAPGKGLEWVSDISGIGSNTYYADSVKGRFTISRDNSDNTLYLDMSSLRAEDTARYYCAKDRKRSGWYEQWGQGTLVTVSS

SEQ ID NO: 178 - DNA, 357 bp, Homo sapiens
  V_region 91..105: note = complementarity determining region (CDR) VH-CDR1
  V_region 148..198: note = complementarity determining region (CDR) VH-CDR2
  V_region 295..324: note = complementarity determining region (CDR) VH-CDR3
  source 1..357: mol_type = other DNA
  CDS 1..357: note = NI-302.72F10-PIMC VH variable heavy chain (VH) sequence
gaggtgcagctggtggagtctgggggaggcttcgtacagcctggggggtccctgagactctcctgtgcagcctctggattcaacttcggcagttatgccatgagctgggtccgccaggctccagggaagggactggagtgggtgtcagatatcagtggtattggtagtaacacatactacgcagactccgtgaagggccgtttcaccatttccagagacaattccgacaatacgttgtacctggacatgagcagcctgagagccgaggacacggccagatattactgtgcgaaggatcgaaagcgcagtggctggtacgaacagtggggccagggcaccctggtcaccgtctcctcg

SEQ ID NO: 179 - protein, 119 aa, Homo sapiens
EVQLVESGGGFVQPGGSLRLSCAASGFNFGSYAMSWVRQAPGKGLEWVSDISGIGSNTYYADSVKGRFTISRDNSDNTLYLDMSSLRAEDTARYYCAKDRKRSGWYEQWGQGTLVTVSS

SEQ ID NO: 180 - DNA, 321 bp, Homo sapiens
  V_region 70..102: note = complementarity determining region (CDR) VK-CDR1
  V_region 148..168: note = complementarity determining region (CDR) VK-CDR2
  V_region 265..291: note = complementarity determining region (CDR) VK-CDR3
  source 1..321: mol_type = other DNA
  CDS 1..321: note = NI-302.72F10 VK variable light-kappa chain (VK) sequence
gaaattgtgatgacacagtctccagccaccctgactttgtctccaggggaaagagccaccctctcctgcagggccagtcagagtattagcgcctacttaggctggtatcaacaaaaacctggccaggctcccaggctcctcatctatgatgcatccattagggccactggcattccagacaggtttagtggcagtgggtctgggacagacttcactctcaccatcagcagcctagagcctgaagattctgcagtttattactgtcaccagcgtagcaagtggcctcttactttcggcggagggaccaaggtggaaatcaaa

SEQ ID NO: 181 - protein, 107 aa, Homo sapiens
EIVMTQSPATLTLSPGERATLSCRASQSISAYLGWYQQKPGQAPRLLIYDASIRATGIPDRFSGSGSGTDFTLTISSLEPEDSAVYYCHQRSKWPLTFGGGTKVEIK

SEQ ID NO: 182 - DNA, 321 bp, Homo sapiens
  V_region 70..102: note = complementarity determining region (CDR) VK-CDR1
  V_region 148..168: note = complementarity determining region (CDR) VK-CDR2
  V_region 265..291: note = complementarity determining region (CDR) VK-CDR3
  source 1..321: mol_type = other DNA
  CDS 1..321: note = NI-302.72F10-PIMC VK variable kappa-light chain (VK) sequence
gaaattgtgctgactcagtctccagccaccctgactttgtctccaggggaaagagccaccctctcctgcagggccagtcagagtattagcgcctacttaggctggtatcaacaaaaacctggccaggctcccaggctcctcatctatgatgcatccattagggccactggcattccagacaggtttagtggcagtgggtctgggacagacttcactctcaccatcagcagcctagagcctgaagattctgcagtttattactgtcaccagcgtagcaagtggcctcttactttcggcggagggaccaaggtggaaatcaaa

SEQ ID NO: 183 - protein, 107 aa, Homo sapiens
EIVLTQSPATLTLSPGERATLSCRASQSISAYLGWYQQKPGQAPRLLIYDASIRATGIPDRFSGSGSGTDFTLTISSLEPEDSAVYYCHQRSKWPLTFGGGTKVEIK

SEQ ID NO: 184 - DNA, 378 bp, Homo sapiens
  V_region 91..105: note = complementarity determining region (CDR) VH-CDR1
  V_region 148..198: note = complementarity determining region (CDR) VH-CDR2
  V_region 295..324: note = complementarity determining region (CDR) VH-CDR3
  source 1..378: mol_type = other DNA
  CDS 1..378: note = NI-302.4A6-VH variable heavy chain (VH) sequence
gaggtgcagctggtggagtctgggggaggcttggtacagcctggggggtccctgagactctcctgtgcagcctctggattcacctttagcgcttatgccatgagctgggtccgccaggctccagggaaggggctggagtgggtctcaactattagtggtagtggtggtagtacatactacgcagactccgtgaagggccggttctccatctccagagacaactccaaaaacaccctgtatctgcaaatgaacagcctgagagccgaggacacggccgtatatttctgtgcgaaagttaccacggaactctacggtgctaactcctactactactacatggacgtctggggcaaagggaccacggtcaccgtctcctcg

SEQ ID NO: 185 - protein, 126 aa, Homo sapiens
EVQLVESGGGLVQPGGSLRLSCAASGFTFSAYAMSWVRQAPGKGLEWVSTISGSGGSTYYADSVKGRFSISRDNSKNTLYLQMNSLRAEDTAVYFCAKVTTELYGANSYYYYMDVWGKGTTVTVSS

SEQ ID NO: 186 - DNA, 321 bp, Homo sapiens
  V_region 70..105: note = complementarity determining region (CDR) VK-CDR1
  V_region 151..171: note = complementarity determining region (CDR) VK-CDR2
  V_region 286..291: note = complementarity determining region (CDR) VK-CDR3
  source 1..321: mol_type = other DNA
  CDS 1..321: note = NI-302.4A6 VK variable light-kappa chain (VK) sequence
gaaattgtgttgacacagtctccaggcaccctgtctttgtctccaggggaaagagccaccctctcctgcagggccagtcagagtgttgtcagcaggtatttagcctggtaccagcaaaaacctggccaggctcccaggctcctcatctatggtgcatccagcagggccactggcatcccagacaggttcagtggcagtgggtctgggacagacttcactctcaccatcagcagactggagcctgaagattttgcaatgtattactgtcagctgtatggtaactcacagacgttcggccaggggaccaaggtggagatcaaa

SEQ ID NO: 187 - protein, 107 aa, Homo sapiens
EIVLTQSPGTLSLSPGERATLSCRASQSVVSRYLAWYQQKPGQAPRLLIYGASSRATGIPDRFSGSGSGTDFTLTISRLEPEDFAMYYCQLYGNSQTFGQGTKVEIK

SEQ ID NO: 188 - DNA, 375 bp, Homo sapiens
  V_region 91..105: note = complementarity determining region (CDR) VH-CDR1
  V_region 148..198: note = complementarity determining region (CDR) VH-CDR2
  V_region 295..342: note = complementarity determining region (CDR) VH-CDR3
  source 1..375: mol_type = other DNA
  CDS 1..375: note = NI-302.12H2-VH variable heavy chain (VH) sequence
gaggtgcagctggtgcagtctgggggaggcttggtacagcctggggggtccctgagactttcctgtgaagcctctggattcacctttagcaactatgccatgggctgggtccgccaggctccagggaaggggctggagtgggtctcagtaattagtggtactggtggtagcacatactacgcagactccgtgaagggccggttcaccatctccagagacaattccatgaacacgctgtatctgcaaatgaacagcccgagagccgacgacacggccgtatattactgtgcgaaagatctgaggaagattagcggtcctttatactactacggtatggacgtctggggccaagggaccacggtcaccgtctcctcg

SEQ ID NO: 189 - protein, 125 aa, Homo sapiens
EVQLVQSGGGLVQPGGSLRLSCEASGFTFSNYAMGWVRQAPGKGLEWVSVISGTGGSTYYADSVKGRFTISRDNSMNTLYLQMNSPRADDTAVYYCAKDLRKISGPLYYYGMDVWGQGTTVTVSS

SEQ ID NO: 190 - DNA, 375 bp, Homo sapiens
  misc_feature 91..105: note = V_rehion - complementarity determining region (CDR) VH-CDR1
  misc_feature 148..198: note = V_rehion - complementarity determining region (CDR) VH-CDR2
  misc_feature 295..342: note = V_rehion - complementarity determining region (CDR) VH-CDR3
  source 1..375: mol_type = other DNA
  CDS 1..375: note = NI-302.12H2-PIMC VH variable heavy chain (VH) sequence
gaggtgcagctggtggagtctgggggaggcttggtacagcctggggggtccctgagactttcctgtgaagcctctggattcacctttagcaactatgccatgggctgggtccgccaggctccagggaaggggctggagtgggtctcagtaattagtggtactggtggtagcacatactacgcagactccgtgaagggccggttcaccatctccagagacaattccatgaacacgctgtatctgcaaatgaacagcccgagagccgacgacacggccgtatattactgtgcgaaagatctgaggaagattagcggtcctttatactactacggtatggacgtctggggccaagggaccacggtcaccgtctcctcg

SEQ ID NO: 191 - protein, 125 aa, Homo sapiens
EVQLVESGGGLVQPGGSLRLSCEASGFTFSNYAMGWVRQAPGKGLEWVSVISGTGGSTYYADSVKGRFTISRDNSMNTLYLQMNSPRADDTAVYYCAKDLRKISGPLYYYGMDVWGQGTTVTVSS

SEQ ID NO: 192 - DNA, 324 bp, Homo sapiens
  V_region 70..105: note = complementarity determining region (CDR) VK-CDR1
  V_region 151..171: note = complementarity determining region (CDR) VK-CDR2
  V_region 268..294: note = complementarity determining region (CDR) VK-CDR2
  source 1..324: mol_type = other DNA
  CDS 1..324: note = NI-302.12H2 VK variable light-kappa chain (VK) sequence
gaaattgtgttgacgcagtctccaggcaccctgtctttgtctccaggggaaagagccaccctctcctgcagggccagtcagagtgttagcagcggctacttagcctggtaccagcagaaacctggccaggctcccaggctcctcatctatggtgcatccaccagggccactggcatcccagacaggttcagtggcagtgggtctgggacagacttcactctcaccatcagcagactggagcctgaagattttgcagtgtattactgtcagcactatggtgcctcatcgtacacttttggccaggggaccaagctggagatcaaa

SEQ ID NO: 193 - protein, 108 aa, Homo sapiens
EIVLTQSPGTLSLSPGERATLSCRASQSVSSGYLAWYQQKPGQAPRLLIYGASTRATGIPDRFSGSGSGTDFTLTISRLEPEDFAVYYCQHYGASSYTFGQGTKLEIK

SEQ ID NO: 194 - DNA, 363 bp, Homo sapiens
  V_region 91..105: note = complementarity determining region (CDR) VH-CDR1
  V_region 148..198: note = complementarity determining region (CDR) VH-CDR2
  V_region 295..330: note = complementarity determining region (CDR) VH-CDR3
  source 1..363: mol_type = other DNA
  CDS 1..363: note = NI-302.8M1-VH variable heavy chain (VH) sequence
gaggtccagctggtgcagtctggggctgaggtgaagaagcctggggcctcagtgaaagtttcctgcaaggcatccggatacaccttcaccatctactatatgcactgggtgcgacaggcccctggacaagggcttgagtggatgggaggaatcagcccgagtggtgcccacacaatgtacgcacagaatttccagggcagagtcaccgtgaccagggacacgtccacgagcacagtctacatggagctgagcagcctgagatctgaggacacggccgtgtattactgtgcgagagggagcacggtgactaactatcgaccctttgactactggggccagggaaccctggtcaccgtctcctcg

SEQ ID NO: 195 - protein, 121 aa, Homo sapiens
EVQLVQSGAEVKKPGASVKVSCKASGYTFTIYYMHWVRQAPGQGLEWMGGISPSGAHTMYAQNFQGRVTVTRDTSTSTVYMELSSLRSEDTAVYYCARGSTVTNYRPFDYWGQGTLVTVSS

SEQ ID NO: 196 - DNA, 363 bp, Homo sapiens
  V_region 91..105: note = complementarity determining region (CDR) VH-CDR1
  V_region 148..198: note = complementarity determining region (CDR) VH-CDR2
  V_region 295..330: note = complementarity determining region (CDR) VH-CDR3
  source 1..363: mol_type = other DNA
  CDS 1..363: note = NI-302.8M1-PIMC VH variable heavy chain (VH) sequence
caggtgcagctggtgcaatctggggctgaggtgaagaagcctggggcctcagtgaaagtttcctgcaaggcatccggatacaccttcaccatctactatatgcactgggtgcgacaggcccctggacaagggcttgagtggatgggaggaatcagcccgagtggtgcccacacaatgtacgcacagaatttccagggcagagtcaccgtgaccagggacacgtccacgagcacagtctacatggagctgagcagcctgagatctgaggacacggccgtgtattactgtgcgagagggagcacggtgactaactatcgaccctttgactactggggccagggcaccctggtcaccgtctcctcg

SEQ ID NO: 197 - protein, 121 aa, Homo sapiens
QVQLVQSGAEVKKPGASVKVSCKASGYTFTIYYMHWVRQAPGQGLEWMGGISPSGAHTMYAQNFQGRVTVTRDTSTSTVYMELSSLRSEDTAVYYCARGSTVTNYRPFDYWGQGTLVTVSS

SEQ ID NO: 198 - DNA, 321 bp, Homo sapiens
  V_region 70..102: note = complementarity determining region (CDR) VK-CDR1
  V_region 148..168: note = complementarity determining region (CDR) VK-CDR2
  V_region 265..291: note = complementarity determining region (CDR) VK-CDR3
  source 1..321: mol_type = other DNA
  CDS 1..321: note = NI-302.8M1 VK variable light-kappa chain (VK) sequence
gacatccagatgacccagtctccatcctccctgtctgcatctgtaggagacagagtcactatcacttgccgggcgagtcaggacattagcaattatttagcctggtatcagcagaaaccagggaaagttcctaaactcctgatctttgctgcatccactttgcaatcaggggtcccgtctcggttcggtggcagtggatctgggacagatttcactctcaccatcagcagcctgcagcctgaagatgttgcaacttattactgtcaaaactataacagtggccctccgcctttcggccctgggaccaaagtggatatcaaa

SEQ ID NO: 199 - protein, 107 aa, Homo sapiens
DIQMTQSPSSLSASVGDRVTITCRASQDISNYLAWYQQKPGKVPKLLIFAASTLQSGVPSRFGGSGSGTDFTLTISSLQPEDVATYYCQNYNSGPPPFGPGTKVDIK

SEQ ID NO: 200 - protein, 10 aa, synthetic construct
  REGION 1..10: note = Epitope recognized by NI-302.64E5
PQPPPQAQPL

SEQ ID NO: 201 - protein, 10 aa, synthetic construct
  REGION 1..10: note = Epitope recognized by NI-302.7D8
QQQQQQQPPP

SEQ ID NO: 202 - protein, 13 aa, synthetic construct
  REGION 1..13: note = Epitope recognized by NI-302.72F10
PPPGPAVAEEPLH